European Patent Application EP 4 368 176 A1, published May 15, 2024. Title: Agent for reducing nephrotoxicity. Applicant: NIPPON SHINYAKU CO., LTD. The sequence listing filed with the application follows.

SEQUENCE LISTING (11 sequences)

SEQ ID NO: 1 - DNA, 22 bp, synthetic construct
  misc_feature 1..22: note = Synthetic
  source 1..22: mol_type = other DNA
gctcggcatcagagggagaccg

SEQ ID NO: 2 - DNA, 20 bp, synthetic construct
  misc_feature 1..20: note = Synthetic
  source 1..20: mol_type = other DNA
ctcggcatcagagggagacc

SEQ ID NO: 3 - DNA, 17 bp, synthetic construct
  misc_feature 1..17: note = Synthetic
  source 1..17: mol_type = other DNA
cggcatcagagggagac

SEQ ID NO: 4 - DNA, 20 bp, synthetic construct
  misc_feature 1..20: note = Synthetic
  source 1..20: mol_type = other DNA
ccttggctcggcatcagagg

SEQ ID NO: 5 - DNA, 21 bp, synthetic construct
  misc_feature 1..21: note = Synthetic
  source 1..21: mol_type = other DNA
catcagagggagaccgtgtaa

SEQ ID NO: 6 - DNA, 21 bp, synthetic construct
  misc_feature 1..21: note = Synthetic
  source 1..21: mol_type = other DNA
ctcgtgcatcagagggagacc

SEQ ID NO: 7 - DNA, 19 bp, synthetic construct
  misc_feature 1..19: note = Synthetic
  source 1..19: mol_type = other DNA
ctcgcatcagagggagacc

SEQ ID NO: 8 - DNA, 25 bp, synthetic construct
  misc_feature 1..25: note = Synthetic
  source 1..25: mol_type = other DNA
aggagggcagcgaactcctggttgt

SEQ ID NO: 9 - DNA, 25 bp, synthetic construct
  misc_feature 1..25: note = Synthetic
  source 1..25: mol_type = other DNA
gtggttgagccagaagctgggaatt

SEQ ID NO: 10 - DNA, 25 bp, synthetic construct
  misc_feature 1..25: note = Synthetic
  source 1..25: mol_type = other DNA
gttgcctccggttctgaaggtgttc

SEQ ID NO: 11 - DNA, 134937 bp, Homo sapiens
  source 1..134937: mol_type = genomic DNA
gatctttggtttgctttcccaacttatattgtgaactgccttctcttcatcccaacattcctgatgttgctgtgtctcagtttacagatgttaaggaacttataatcaaaactgtattaagctcggcaagagatgagccctctggtcctgcacgatgtgtagcactttgtagtttaggtatttggatttgtgaagaactagtccatgagtctcatcatcctcaaattaaggaagctctgaatgtgatttgtgtttccttaaagtttactaataaaacagtagcccacgtagcttgtaacatgcttcacatgctggttcattatgtacctagacttcagatttaccagcctgattctcccttgaaaattattcagatcctaatagctaccatcacccatcttttaccaagtacagaggcttcatcttatgaaatggacaagaggttggtagtatctttacttctctgccttctggactggatcatggccttacctctaaagacactgctccaaccatttcatgctacgggagcagaaagcgataaaacagaaaaatctgttctcaattgcatttataaggttttacatgggtgtgtttatggagctcagtgttttagcaatccaaggtattttcccatgagcctctctgatttggcatctgtagattatgatccttttatgcatttggaaagtctgaaagagcctgagcctctgcgctctcctgactcagaacgatcttctaaactccagccagtaacagaagtgaaaactcaaatgcagcatggattaatctctatagcagcccgcactgttattacacatctggtaaatcacctgggccattatccaatgagcggtggtcctgctatgctaacaagtcaggtgtgtgaaaatcacgacaatcattacagtgaaagtactgaactttctcctgaactctttgagagtccaaatatccagttctttgtgttaataatacaaccttagtgtcctgtatccagatcagatcagaagagaatatgcctggaggaggtttatctgctggccttgcatcagccaattcaaatgtcagaatcatagtacgtgatctctctggaaaatattcatgggattctgctatactgtatggcccacctcctgtaagtggcttgtcagaacctacatctttcatgctttcattgtctcaccaagagaagccagaagagcctccgacatctaatgaatgcttagaagatataaccgtaaaagatggactttccagtttaaaagatttagagaaactgtaccaacttgggatacaataagagatgaagaagatgctcttgatgaactcttgcagtatttgggtgttactagtcctgaatgcttacagagaactggaatctcacttaatattcctgctccacaacctgtgtgcatttctgaaaaacaagaaagtgatgttattaatgctatccttaagcaacatacagaagaaaaagaatttgttgagaagcactttaatgacttaaacatgaaagctgtggaacaagatgaaccaatacctcaaaaacctcagtcagcattttattattgcagattgcttcttagtatattgggaatgaattcctgggacaaacggaggagctttcatctcctgaagaaaaatgaaaagctacttagagaacttaggaacttggattcaaggcagtgccgagagacacacaagattgcagtattttatgttgctgaaggacaagaagacaaacactccattctcaccaatacaggaggaagtcaagcatatgaagattttgtagctggtcttggttgggaggtaaatcttacaaaccattgtggttttatgggaggactacaaaaaaacaaaagcactggattgaccactccatattttgctacctctacagtagaagtaatatttcacatgtcaacaagaatgccttctgattctgatgattctttgaccaaaaaattgagacatttgggaaatgatgaagtgcacattgtttggtcagagcatactagagactacaggagaggaattattcccacagaatttggtgatgtccttattgtaatatatccaatgaaaaatcacatgttcagtattcagataatgagaaaaccagaggttcccttctttggtcccctttttgatggtgctattgtgaatggaaaggttctacccattatggttagagcaacagctataaatgcaagccgtgctctgaaatctctgattccattgtatcaaaacttctatgaggagagagcacgatacctgcaaacaattgtccagcaccacttagaaccaacaacatttgaagattttgcagcacaggttttttctccagctccctaccaccatttaccatctgatgccgatcattaaatatcagttctgtttatctgaaggctcctacccagagattctacccagtgaaactcccacagcagcgcaggtagatggggctgacctggcctctccaatgtctcctcgaactagcaaaagccgcatgtccatgaagctgcgtcgttcctctggctcagccaataaatcctaaggagacaagcagcccagcagtgatcagcagtagccaccttagcatgaacatagggttaaccctttcaggccttcatgtctgccataacatgcatgtttcttcctgtacatttatttgagaaaacactggatttaaataattttaaataatttgtagcttaatattaaagatttaagttatttattgtttcatttttttcccacaatccaagctgccatattttgagggcagggggagttttattctacaccctttaccttcctagataattatgtctaagtagttttatctttaatttcatggttaactgtgagccaaaatacaattggacaattagtctcattatttattgtgctccattgcaactttatggttcaataaatatataattttttacaaatgtaaaattttacatttaagcatttgtaaagttacagcaaaagatgtacctgttaatacacagaatgtgtacagattatttgttatgacaataaaacactcaaaataaatggtctttagcatctcaaattccaactgaaatcattttagtattaactcttcttcccaaagcaatgtctcatttcttggctgtgcaggtgatgccatgttatatccaataactagaaaaatcactgtgctgaacttttatgtttagcttccaagtatttttctaatgttttgcatttcaagtggtatcactgttaaatgccatttgttttcagattgtggccttttattattggctgctagatcctggtgtttctatgttcttttttaagcaccaaaaagaagatggggaagaaaagaaggaaaattttctgatataaatatgttgttcaaattatgagtactatttaaaaaagaaaaaggaacctaacccaggagtctaagttaaatctaatattgttaatactgaacttgcaggtccaggttggtatacattccaccctctagaagtattttcttacagtagataagctgctcacattttgttttgaatgggcatctcctgaggaaatgtagcatgatattggtactaactgcatgtgtaaatacatcatactggcaagccgtaaaatataaattatgtatcattcacgtagtatctataatttgtaacagtggggggaaaagatgacatggtatttaataatacaataaaaatattcttatcaaaaaaaaaaaagaaaagaaaaccagcacaagacaaggatgccctctctcaccactcctactcaacatagtattgaaagttctgaccagggcaatcaggcaagagaaagaaataaagcgtattcaaataggaagagaggaagtcaaattgtctctgtttgcagatgacatgattgtatatttagaaaaccccatcttttcagcccaaaatctccttaagcttataagcaacttcagcaaagtctcaggatacaaaatcaatatgcaaaaatcacaaacattcctataccccaatgacaggcaaacagagagccaaatcatgagtgaactcttattcacaattgctacaaagagaatacgtaggaatacaacttacaagggatgtgaaggacatcttcaaggagaactacaaaccactactcaaggaaataagggaggacacaaacaaatggaaaaacattccatgctcatggataggaataatcaatatcgtgaaaatggccatactgctcaaagtaatttatagattcaacgctattcccatcaagctaccattgactttcttcacagaattggaaaaagctactttaaacttcatatggaaccgcccgcatagagaagacaatcttaagcaaaaagaacaaagctagaggcatcatgctacctgacttcaaactatactacaaggctacagtaaccaaaacagcatggcactggtaccaaaacagatacatagaccaatggaagagaacagagacctaagaaataaaaccacacatctacaaccatctcatctttgacaaacctgacacaaacaagcaatggggaaaagattccctatttaataaatggtgttgggagaactggctagctatgcagaaaactgaaactggaccccttccttacaccttacacaaaaatcaactcaagatggattaaagacttaaagataagacctaaaaccataaaaatcctggaagaaatcctaggcaataccattcaggacataagcatgggcaaagacttcatgtctaaaataccaaaagcaatggcaacaaaagccagaattgacaaatggaatctaattaaactaaagagcttctgcacagcaaaagaaactgtcatcagagtgaacaggcaacctacagaatgggagaaaatttttgcaatctatccatctgacaaagggctaatatccagaatctacaaagaacttaaccaaatttacaagaaaaaaacaaccccatcgaacagtgggcaaaggatatgaacagacacttatcaaacatatgctaacaaagatattaaaaaaaatgctcatcatcactggtcattagagaaatgcaaatcaaaaccaccatgagataccatctcacgccagttagaatggcgatcatgaaaaagtcaggaaacaacagatgctggagaggatgtggagaaataggaactgttctacactgttggtgggagtgtaaattaattagttcaaccattgttgaagacagtgtggcgattcctcaaggatctagaactagaaatatcatttgacccagcaatcccattactgggtatatacccaaaggatttataaatccttctactataaagtcacatgcacacatatgtttatcgggtcactattcacaacagaaagccttggaaccaattcagatgtccatcaatgatagactggataaagaaaatgtggcacatatacaccatggaatactacacagccataaaaaaggatgagttcatgtcctttgcagggacactgatgaagctggaaaccatcattctcagaaactatgacaagaacagaaaaccaaacgccacgtgttctcactcataagtgggagttgaacaatgagaacgcgtggacacagagaggggaacatcacacatggggcctgtcggggtgggggtctagaggtggaatagcattaggagaaattcctaaggtaggtgaccggttgatgagtgcagcaaaccaccatgacacatgtatacctatgtaacaaaactgcacattctgcacatgtaccccagaactttaagtataataatattaaaaaaaaaagagaaaaaaaatcacacacaggatttgggtctggagcaagagtcctgagacaggttatttaacctgttagaatttgggggactttcattaaagaagtggtatttaggccggttcttgagcaagtgggaaaatgtatggttgttagacttgcagtgaaaggcggaacagccatagcaaaggcactgaagcagatggtgtgagtttaaacaacattttgactggtatatttagctatatagtgctctctaggagttagaaggctagaaaggcagattaggactaaatcaagaaccagaatgtcatgctaagtcgtttgtaagtagtatagaagtaaatgatgatttttaaatagaggaatcagagtaagctttatcttgtaataatgaaaaagatgaattggacagtaaagaaattatctgggaagctggtaaaacagtccagactagaggtagctgaagaggcttacttaaattcagatagttaagtggccagggtgtcctttagggaagtggggtgagggaggggatgggaggagatcatgcttgacataaaacttattataagttgtttcttgcaaaagtgacttaggattggaagtctggaatgctgcaatggaagagttttccttacttaacttttctctgaaattaaactgccaatgtcaatagttatgtctgtttttcttttctccatgcttccctttatttctttactactggtaagttacaaatttttaaaaattgtttttctgttatcaaaagagctcttaatacattttgaagcagtgctaagtgaaatttttctctttatttgtatgacgttcactttctatttgttgccctgagttacttgggaaatatttttcagaatgcatgtttcctctcagcagacactctgaccaccagttggggaggcaaactatcagtgtattttgaaaaagtttcctgattgtttctgaatctgctgtgccttttcaattgacaatcattgatttattacaaaatgccaaaggcctttgttttttcaatttagtactttggctcaggaagatacaggtgttccttaattgatagtatcacatactctactcagctgagctcattctagtcagatattgtacacctactctgtactgaggatacagagatgagatgtggatcctagcaacagttagttcccttccctcagctactccatagccaagttcctcacttgccgtaaccaataagcgctaagcatgccgtatgatagatttgtaaaacctgtcttttcatcacccttttaatccctactccttgatagaggagttttgctttgttttacctcagtggctcctagcccagatgaacagcaaaatcctgaaattcttaatttaaaaaccagacatgtgtttctcaagcctaccctccagtatctgatttagtagtttatggtaagtcctggtaatttgcatttttaaaaggtccccaagtgattctgatgtgcagctgggttgaagaaccactggtttggttcatttaattcctcctcactcctgattacacatttactttaacctctcctctcctttcatttcattcttacctagttacccaaaacaaaatcttgttgactttctttgctctgtttcttagctgaatagcaaccatagtcatgattgttaatggtaagatagtactagcaatactaaaaagcactggggcttaaagtgaagttagatataatgaagagctagtgttctcaggttattgtatcccatcttccttctctagttacaaaagtaatttttacaaatactgacgtgattaattaaaactgtgttcatttttgtatagttaccaatatttgctgttgaataacttgggtggaggaagattaatgtgcagtcaatttatgaattggtgacttgatgaattgggtaatatttggtgacctctgcactcattttttctaggggagaatgtactttcatttcagataatgtcacatgaacttttggagaataactgtcaaccacaggaagttcttttattatataggtgttctggagacctaaaagcttttttgttataatttatataccgtgttgaaacaattttactttcgccctcttccttttcatgtcttcttttaatgttgcatctaaaacattgttttttcacacctctttttaagaaaagcaacagcatggtttctttcatgaaatgtttccagaagcctgatccaaaaagagaaaagtatagctggttaaaggagggaggaagccctaaatctggcttcttcccagagtacctctgtggcatctgtggattcccttgagttcagcacatggtttaaacaccattgatttcaagagtctttgcccctcacaagatcaggaaaatagagctgcatgtactatttttttaaactttgaggcaaatgtaatgttatcttttctcctgagcttaagataaagcttttgaaaacatacagaccttttgtgatcgggcttttaacattctctatcagcttgtataaaatgaatcagaaagaaaattatgatacagttcttttttcctgagttatcagttgacaatgtttgcagttttactttcttactatactagttaatgactcttacaagtattgtataagatcagcttagaatacatgttcatctcaaaccttgaagaagtgaaaacatatatttttggtattcagaataaaaagtataaatgtttaataatttttatttgtttctatccttcattttggagatctcaacaactattctggaattttcccccctcacgttctgttttgctgtccccgtacccaatagcaagaaactactgcctaccttagcacaagtttcacagaaattttaatctacctatccacattcagctttgctcatgctatctgttcaaacagaacttatagtcagtttttagttgtctttttaaagaaacatctttacacaaaggacctttgaaatcccttgggaagaattaaactaagtcatgtgagtgttgtagttctagacttacacttttgctacttaatattatacactaaaaaggagacagttgaagtggtcctgagttctttgaaattgtctaataagtctgatttctgacagcaagacatttaaataatgcagaatgaagtcactgaatcatatgaaatgaatcatatgaaatgactttaagttttatctgtattcttgctttgccatcagggatttctagtctagtattggtagcttatattaaaatctactcagttgatcttttcttaggaagaaaatttctagtgctatgttagaaaaaagtgtttttatttctaactagtggtgagaatatagttatccccatatcccccaaatacttttaggataatcttgaccaaaaaatcttttgttaaatgcagtaattcaatataattaaaatgtttttgaaaacatctttgggactgaatctgttttgagtttttgaatgttagtaaacatcccaatactccagttttccatatatcatataatttgatataagaggaagtcaaggtggatcttgtctatttgagtaggagaaatgcttgataatacttgatattatcctgtgcaaggatttggataattgccatttccatcttttttttttttttttgagatggcgtctagccctgttgcccaggctggagtgcagtggcgccatctcggctcactacaacctctgcttcctgggttcaggcaattctcctgcctcagcctcccgagtagctgggattacaggcacccacaaccacacccagctaatttttgtatttttagtagaaacggggtttcactgtgttgcccaggctggtctcgaactccagacttcgagatccacctgtcttggcctctcaaattgctgagattagaagcatgagccaccgcgtgcagccccccgtccctttttttttaagacagagttttgctcttgttgcctaggctggagtgcaatggtgcaatcatggctcacccgcaacctctgactcctgggttcaagcgattctcctgcctcagcctcccgagtagctgggattacaggcatgtgccaccacgccctactaattttgtatttttagtagagatggggtttctccacgttagtcaggctcgtctcgaactcccgacctcaggtgatcctcctgccttggcgcctcccaaagtgctgggattacaggtgtgagccaccgtgcctggccgccatttctatttttaagaaggtaagattcagagcaaaaatactcactgcttataaaaagagttatttagtcaggattataagaagaaacctatttttgccttcatttaactgcaaaaaaatgtaagctgtaactcattatctttcttgagttcttttttttctttagtaaatcttgtcacattttagcattgtttcttatttcagccgtgtattctttgtataagccttgctcagtctgcatgccattagtgttttcagcctgctttgtattgatagcttcttacatttcagtgtttataattgacagcgctctttaattaactagttcagatcaaattgaatggtgttatttctataacataattagaaatcttttcagaggttccttccatgatttctagttttagtttatgaaacatttacagtataaaatatttgtttttcttttttctttttgtttatatagaagtggtacaccatccccaaaacgaacatctgtaggctccaggccaccagcagtaagaggcagtagagatcgttttactggagaatcatacacagtgctgggtaggacaaaacataattgtttttcattatctcagattaaaggcatcacaatcacactggtggactttccactcaaagtgactgcctgtatattgaataaatctttgcaagaaatttctcccaattgaagcctaattactttggggagttttcagattgtcttattattattgatacttttaaaactctacttcagcttacgtagtgttcccacatctttatatataagccgggaggggggatagtaaggaagaaaacctctgaagcgttttatattcaagaatagtactaaacgtaaaggtaaagttagagcaggtactcagcatttaatgtctgtgtgttaacatgattattcttataggaaaagtacttgaataaaaatttttgtgtctttttttgggacgagtggtaggtaaaactgtgtgactcataaggaagagatgagtcaaatctacctttctgatcttttgtaggagacactgctattgaaagtggacaacattattgggaggtcaaggcccagaaggattgtaaatcctacagtgtgggagtagcatacaaaacgttggggaaatttgaccaattgggaaagacaaacactagttggtgtatccatgtcaacaactggctacaaaacacatttgcagcaaagcataataataaagtcaaagctttggatgttactgttcctgaaaaaataggtgtattttgtgattttgatgggggtaagtttattttctcgtaggttatttcatcatagttgcttgcatttcagtacctttcactggtaatcatctatacaggatttccattagtattgtgggaaggacattttgatcaggtaggcttttgattgcaatcataatctcaattctagaattgactggaatggtatatgtgatgtctgcctggagccctataaaagcactcatttataatatactaagtctgaaagattttgctaattttagtcttcagcactaacatttcttctgtccattttaattccttccttaccatgttttattacctacctctaaagagtgatagtcaaaattttctagttgaagtagatcttagaaattacccaacccaggatgaataccccattttacatgatgtgattattacacattgcatgcctatatgaaagcatctcatatactgcgtaaacatacacacctactatgtacctacaaaaattaaaaaaaaattcaagaagataccagagccatattttctactatcctagtaaacataagctatacagcaaatatttactgtgccaaaccgcatcacacttgaaacaaatggaatgttcttaattttcaagttgctgtctttaaaaatattcttcagaatgactcatgatatctttagaggggccaaaggggtttcccctcaatatcagaatttctttacttacaaaattattaacacagtgtagtctaatccaaaaaagaaaagaaattactccatctgccacacagtatacagttcttagtacactatctctgcaggtagttgccacttatgtgcctgaagaacttttaatgtgaagtttactgtcttagaaagcagcctgtttcattgttggacagctcttggttagaagatttttcttaagttgactcacattgtttcccttaaattttcccatctgaataaacacagaattacgtttcctcactcatgttcacacgataatcctttattaaaaactttcttgccctgtttttccagaccatatattctgttattagctgcccctgttaaaatttaatttttccaagtctttataatctcctatggctgtctagtatgtcagtgtttttcttaaaggttggtcttagagtggaacacatgacctctgaccagcaaaggacagtaatttggctatgctatttctaatagtatgacttagcactgctgatcaatattgagcttgtagctaccctaatccattagatcttttttcacggcattatgtcaaattgtctttttcttttgttaggcagtttatggttttggttttttttgttttgttttgttttgtttttgagacagagtcttactctgttgtccaggctggagtgcagtggctcaatctcagctcactgcaacctctgcctcccatgttcaagcgactctcctgcctcagcctcctgagttagctgggattacaggtgcatgccaccacgcctggctaatttttgtatttttagtagagacggggtttcaccatgctggccaggctggtctcaaactcctgacctcaagtgatccacctggctgggcctcccaaagtgcagggattactgccatgagccaccacacccagccagtttatggtttttaaaaataactcaatgttatatgtaatgcaaatgaagactattacatttacccttttttagtttcatcttaatagatttggcccaaatttcccgtcttaaaattatctaaaaatttacttgatatttatattttgaaaaaattttaaagctcattgaattagttatttcataagcatattctctacagtcatctaatgtataataattttgaagatgacataatattgaactaaagtaattccctagatgttttttctccaagttgacacttaagctaataccaaattttattattttagtaatattgtgcccaaataattccatgagctgtcagttaatttactcaaaaaaggagaaaaagtaattttggcttgatttatttttagtgatgacatgttagctttgctgtgttttttgttttttaacttattcaccttgaatcagttaaatcattttcctcaggataaatggcaaatttattagcacacatttttttttcaactaccaagacaacatttgcttcttctctctcctttcccatactctgtgagtccataaaggtagtagtgagatacagtttttagtctagaacataacgtatggcaaggggaagttgtactgtggaataggatcagattctgagagccttgaaaaataataatggactggtcttcagtagtggggaggggtggttctgcatgttttagaacactatagtcataagataattgagttttagaaatattagagagtcagtggttaaagatggaagagatcgaaagcatagcaagcataagacttttcgggaagcagtcttcaagtggtgtagagcaggactgagtctcttgttagctattaagcccttattgcctggctagtgcttttcacatagaaagcccttaataagtgttgagtaactggcaacaagcatctgagcagtggagaattaagaatggatttgacagtgtagaagtagaattcataggacttagtaactaaatacagatcagctgaggacagacagttgaagatgactttgaggttccagccagtgtgatcaagaggatgacagtgtcaacaggatagggaacatagagttttggggggaaatgaaatgccagcaggataatcatgtggcatgtttagcaagcattttgaaattcagtgctagaattcagcagttaagtagagctgacattaaatatttgagacagcattacagaattgctatggaagattgtacaggacaatatatttaagcattactattctgctgtttactaactttgtgatcatatgtaccgttatgctgtttaccaacttcgagatcaaagtactgggtactttacatacattacctcaaaatattaaacaatctacataataatgtgcataaatattagtttattttatcttcctctttggtggcagttgatttattaaggaagcattatataaagaaaagagagcatggacaaagtggctacatttagaacaggaagaaaaggaggagatggtgaagttatccccagggttatgatacaaaccaagggaatggtcatcagagaagagtttcaagaagtgataacagctgtaaggaggccatttggttggccagtttaggaggtcagacagacagttttttttagggcatgatcctattgaaggatatactgtgaggtgattttaaaaattaacaaagcaggtcaggcatagtggctcatgcttgtaatcctagcactttgggagactgaggtggaggattgcttgagctcaggagttcaagcccagcttatacaaaatagcaagaccccgcctctgttaaaaaaattaacaaaattgaagcagtgatagatatattgtgattttagagactggagtatcagtatcgcatcaggtagatagaagacaaggtttaatagagtaaaccttaaatggtgattagaatttgggcagagaggctggttataggaaaaataaggaggaagaaatggccttggtttacactgggctaatgaaaccatttgttaaataatgatcaaataaggaaatagtttgtattaaataagtcgaatcgtgctagattatagaggtattatagaggtcttgaaaaccaggggaagaaaattggattgggcttttccttaagcatttgtccttctgattttcaagtgagaataattaatccagtcctcatacaaaaattaatgccaacttatatattattactttttgcatgattatgcgttagaattaattaaatgttacaattttttgtataataaattaggctttttttccttcttttttaggtcaactttcattctatgatgcaaattctaaacagttgctatattcctttaagacaaaatttactcagccagtactacctggtttcatggttagtatgttttatatcttatatatacctaacatattttacttggttggcaactttaaggagaatattctatactgtatatttggagaaggagaatattttgttttttcttcatattctcctccatttccccaattcaccctctcccaaatctgtgattgtttttatatatttttggtatattttattgaagtttatgttaatacatgaagtacacaaatcatgtagtttgatgagtttttataggactgcactcatgtgtaactagcacttagaacattacgagaacctcagaagccccctctagtgcccatttccagtccctaatggcccttctccagtgttagcactgtattgacttttaataccctaaatttacttccttttcagttttatataaacagaatcatacagtatctttttgactcaacattatgcttgtgagattaatccatattctatgtggttatagttcattcattctcatagctgtatagttttccattctgtgactatatcaattgatttataaattttaatttagttggatatgtgggtggtttccatttgggggctatacaaatagaactgctatgaatacttttgttcatatcttttgataaatgtatgtgtatatttccattgagtatatacctatgattggggttgctagatcatatcgtatatgtataatcaactgtaaaattgccggttttctgaaatggttggttatgctaatttacaactagcagtatgtaagaatttgagttccttcaaatccttgtcaacacttagtattatcttttaaaaaattttttgtccttctagtggatgatatattacattttggttttaatttgcatttccttgattactagtgctgttgagcacctttttatatatttgttgactatttgggtatatgcttttgtgaactggctattcagatcttttgcttgtatttctattaggttgtcttcgtgtttcttatgggttaatttgtaggctcttcttcactctggctttcctttttccttattggtattgtttgataaacaaaagttaattttgttcagtttatcaattttttcatttacagttagcactttttgtgttctgtttaagaaatcagtatgcacccccaaggtcatgaaaatattcttctaaaagctttaccttgtacatttagatatagactgcatttacaatgcaagtacaatgtagaattgatgtgtttggtatgaagtaaggatctagatacgttctttaattccccatggatatccagttattccaggaccatttattgacaagatcatagtgcagtgtcatctttgtacaaaatattagatgactgtctttgtgtgctatgctgaatatatgtatgcacaccacatagcaattacatcctgtgtaattgcaggtctactcaatttcaggctgaaaagaaaaatttgtttctctgcacaaaataaaacatggttttgaatttatttaagcaaatgttattgctttttccaactcataaccttctgcatcttttcataggttaggttcccgtggggagttgtgggatccagttaaagttaccattactttggctagagcttttcttaaatttggaggctacctctataagtcaagatggtatatttcaaatggaatattttgcatgtatattcttctgtcatcacccctaactgtaacttcccaactataaggagaaagttttcagagtaagagtgggttgaaaatacagtgcttttaaatctcattatccatagtaattatttattccagatactttaatctcttaagtttaaaacaatgctaataaccaggacacctatttttacattaaaagtaagtgattagtgactaaagttattgctcatggaaacataaagatactggaagggagggttgtttctttttcctttttttttttttttaactttgtacaaacctctgccatattacgcatttttggctatttttccaaactggtccatcaaggatgagttgtttaccatgtggaatgcagaaaaattttttccaagacttaggtgtgcttttataaatagtagatttacttttaatttgaatctatctcatgtatgtatgtactgagtttattgtttttcattccaaataatactctaattatattagtatatgtcataagatactgcaagaaattattttaagcttgttaaaattttttttccttcattgaaggcttgcttttattaagtacgttaatgcctattaaatgttttgtgtacaagattaatttttaagtcagttttattgaatttatagtatggtgcagttctgtggtttttagcaaatgcctgcagttgtataaccaccaccataatcaagatatagaacatttccatcaccctagaaaattcctttgtgttcttttatagtggaccgttccacacaaccagccctagctatcagtaaccagttcgtaggccctatagttgtaccttttccaaaacatcgtataaatagaattgtatggtatgtagcctttcgattccgtaccatgctgcatttgaaattcatccatgttgttgtggtgtcagtattctcctttttttcattgctgagtagtgtttcatatatgtatgtatcacagtttattcattcattcaccagttgaaagacacttgggtttttcccagtttggggcagttatgaataaaatcactataagcatttacatatgggattttcccttgggtaaatacctaagagcagtaatagagtagctgtatcacattgaaagtgtatgtttaacttcatggggaactaccaaaatgttttccaaagtggctgtaccattttttgccttcctatcagtgatatgagagttggtcatatccttgccattatttgatattaccagattttttgttgttgttaagccattttaataggtgtgtagtggtatgtcattgtgtttttatttgtagtttcctaatgacaaatgatgtttcatgtccttatttgccattcatataatttatttcaagtatctgttaaaattatttgcttactttttaggacttaattgttttcttatttttttattttactttatttttaagacagggtctcgctctgtcacccaggctagagtacagtggtgcgatcacagctcactgcagtcacaactgcctgggctcaagtgatcctcccaccttagcctcccgagtagctgggattacaggtgcccaccaccatacccggctatttaaaaaatgtttcttgtacagatggagttttgctatattgcccaggctggtctcaaagtcctgggctcaaatgatccaccagccttggccccccaaaatcctggaattacaggcatgagccactgcctggttttcctgtttttaagagttctttataagtttggatgtgaatcctttgtcagatatatgctttgcaaatattttctcctggttatggtttgcattttcattttctgaacatttcagagagaagtttttcattttgttatgaagtccaatttagtaatttttttccctattatgggtaatgctttgcttaactcaaggtcacaaaggttttatgttttcttcttgatttccctttgcatcttcatgttagatattttgagtaaatatttttctaaatcatttaaataatttccaaaaaataatatagtagttttataatcagaaagttgcttttgtattttgggagttatcattactgagcctgttagttttgaaaatttataatgttaattatataattacaaatttcacagttcagtagattctttggtataataatctagttacttagtagatattgaacacttaagggtataattgaaggtgatgatacttaaacaacttctagaatttcccttgctttaagcttgtgtctactattaatatatacggtagttgatgatagtgtcaatgatctgtattttcatattttaattcttttgactgtgtcccaaatcttatgtctcactttattgaattatagctgctctgttcccaagcagttttaattttattttattttttgtttttatttttattatactttaagttctagggtacatgtgcacaacgtgcaggtttgttatatatgtatacatgtgccatgttggtgtgctgcacccattaactcgtcatttaccttaggtatatctcctaatgctatccctctcccctcccccaaccccacaacaggccccggtgtgtgatgttccccttcctgtgtccatgtgttttcattgttcagttcccacctatgagtgagaacatgtggtgtttggtttttgtccctgcgatagtttgctgagaatgatggtttccagcttcatccatgtccctacaaaggacatgaactcatccttttttatggctgcatagtattccctggtgtatatgtgccacattttcttaatccagtctatcattgatggacatttgggttggttccaagtctttgctattgtgaatagtgccgcaataaacatacatgtgcatgtgtctttatagcagcatgacttataatcctttgggtatacacccagtaatgggatggctgggtcaaatggtatttctagttctagatccctgaggaatcgccacactgtcttccacaatggttgaaccagtttactctcccaccaacagtgtaaaagtgttcctgtttctccacatcctctccagcacctgttgtttcctgactttttaatgatcgccattctaactggtgtgagatggtatctcattgtagttttgatttacatttctctgatggccagtgatgatgagcattttttcatgtgtctgttggctgcataaatgtcttttgagaagtgtctgtccatatcctttgcccactttttgatggggttgtttttttcttgtaaatttgtttgagttctttgtagattctggatattagccctttgtcagatgagtagattgcaaaatttttctcccattctgtaggttgcctgttcactctgatggtagtttcttttgctatgcagaagctcttcagtttaattagctcccatttgtcaattttgtcttttgttgccattgcttttggtgtttcagacatgaagtccttgcccatgcctatgtcctgaatggtattgccttggttttcttctagggtttttatggttttaggtctaacatttaagtctttaatccatcttgaattaatttttgtataaggtgtaaggaagggatccagtttcagctttctacatatggctagccagttttcccagcaccatttgttaaatagggaatcctttccccatttcttgtttttgtcaggtttgtcaaagatcagatggttgttgacgtgtggtattatttctgagggctctgttctgttccattggtctatatctctgttttggtaccagtaccatgctgttttggttcctgtagccttgtagtatagtttgaagtcaggtagcgtgatgcctccagctttgttctttttccttaggattgtcttggcaatgtgggctcttttttggttccatattaactttaaagtagttttttcccattctgtgaagaaagtcagtggtagcttgatggggatggcattaaatctataaattaccttgggcagtatgaccattttcacgatattgattcttcctatccatgagcatggaatgttcttccatttgtttgtgtcctcttttatttcattgagcagtggtttgtagttctccttgaagaggtctttcacatcccgtgtaagttggattcctaggtattttattctctttgaagcaattgtgaatgggagttcactcatgatttggctctctgtttgttattggtgtataggaatgcttgtgatttttgcacattgattttgtatcctgagactttgctgaagttgcttatcagcttaaggagattttgggctgagacaatggggttttctagatatacaatcatgtcatctgcaaacagggacaatttgacttcctcttttcctaactgaataccctttatttctttctcctgcctgattgctctggccagaacttccaacactatgttgaataggagtggtgagagagggcatccctgtcttgtgccagttttcaaagtgaatgcttccagtttttgcccattcagtatgatattggctgtgggtttgtcataaatagctcttattattttgagatatgtaccgtcaatacctaatttattgagagtttttagcatgaagggctgtcgaattttggtaaaggccttttctgcatctattgagataatcatgtggtttttgtctttggttctgtttatatgctggattacgtttattggtttgcgtatgttgaaccagcctaagcaaagcagttttatctttcacaaagtcattcacatttatgataagtaatagaacatgggaagtacatctggatattgggatttgcatttttgtcaggagtccttcttaaataattatataagagttcttatagttaacacggtaaggaagaaaacagtggattttactgttaactgaggggtgttagatttttatagtctcaggccatatctcattatcaaaaccaaaagcataagtgggaagtaagttggtgctttgtatgcttcccttggttgtgaaaattagcatcagtaatgataggtaataccttttgcctagattaagccaatgaagtttctcaatttctgcacccctgagttccttctcttgggtgcagcttcagttggttctgctaccaccaagacctcctctggcctctgtggttctaaaataattctgatttagtctttccatttcccctcagctgaaatatgacagttaatgtgtttgagaatgattgatgttcatatgtgtggcattttgcctttgaaatggaaatttaaaaatcactgaaattctagtttgatttgcaatctgacaggtttttttgtcttttcttaggtatggtgtggtggactttctttgagtactgggatgcaggttccaagtgctgtgagaacacttcagaaaagtgaaaatggaatgactggttcagctagcagcctgaacaatgttgttactcaatagtgtctactcagaatacgtttaccctccgtcttgattaggtggccttttctgtgcagttactaatcacaggaatttggtagtagtgaaaatcaggtttgctgtgttctgctttgaggcctggaatcttttatcattaaacacctagtacgaagcatttgcaggaacctactgtgcagtatcatagaagcaagcagataccaagcaaaaaactgatgattgaagagtaaatgggggaaaaggcagtgtttaattaacataaaaactcatttttgtatttcttggattactttgactattctaatgtttaattacatatggtaaccctaaggcctggggagaaaagcttttaaatcttgccttctttcttctgtactttgtctttttaaaatctcattactatctattatttagttctaacacagaagctttaaaaatacatagtcatccaaggttttctaaaaattgaaatcatatgttgggaatggtaaaaaggttttcaaatggtttatttttcctcttttataaataagttttacaaaattttcctcttttgtttattgactagattgtatataattttcttttttccaaaatattgtgataagaaatttctagacacaacagcttaaaatcacccaaatttcagttctttacctactgcactaacaatggcaaggggggtattctttatatgttgccttgtttaactacagttcttttcattccatcactttaggtgatgggtaagatttttgaaagccttatattttttgattttgttgtctagtttaatcctacctttaatagttgtgtttggtaaaattcccacttgaatgtgacactgataataattatgctgatttttagcatctcttataggaatcaaagtttattaaagttacatagaggattgaaaaatgtatatcactcaatttttatctaagaaggataggttataaagggaggtacctaaatactcaaataatgtatatattctttttcataacatatggaatgctttaagcaattgttttgaaaaaaatctgcgtatctttgacttaattggcacatgactttttcaagcagccattcattcagaggtttgttttctctcagtccttttgctacattcactttcttttcaaagaaatgttaattattacaaaaattgacatagatatctttcccaaacttggggtaaaacccatggttatgtggaacataactgttcttaaaaagtcaattataatttgtaactcacatcctttgagctaaactaaattaaaattacagtatttaataattctttgggcatttttaagaggtctgaatttgtatttttcttcatttttgaaactttacatttgttgactttttttcattctcatttaaaatatattgtgctatgataaccaaccttcttccaaggagtgaccattactgcctacatttgcgttgctttctacatagagacttgtataatagtattaatagtagctcattctctctaaaaatttactgcccactgataggatgttttgtttccttgataaaacaaatgtaaatgaggaattttatttgaattggaatattgtttttctagaggacattcatatctgcactattatctgatgacatgttggtaattttaaagactgcaaggcagtttagagaatgaagtaaaccaatagatactcttttgattctccaaagaaatataattttggtttttgttcctcagagagagtttgaaagaaattttcagatgttctgttccctatagagggcctattccaggatctaaatgaatgggaatttataattcctttcatagactcaaacctgaaagcagaaatttttagtagttgagttgctttaagtgaattttaacaaatatgacacagaaaaggtcagatgctgttgtataaaattttttactagtgtgtcttatataattctttcttctcattaattcagtgcctttttcctctaagcatactcttggtccatgccccatgcagtgtcaactgatgtttaagctacagagcattgttgtagtggtgagggccctctgttgcaggggcatggggaaatgcatatattaatcaggggctggaggagtatacatgattcttgtgttcatgttgtcatttgaaactcttcacataaaattttctaatattcatttggaaaacctctccactggagaggtttcatctctgagaggttttgtaataatagtgtaagttcagtaaatccagtccaaattctcatcacatgtattatttgatactaaattttcaattattacttcaaaataagagtctgaggatttcttcttactggcgttcttaaaggtctctaaaattaaagaacaagatgtggttttttgtttaagacgtttttagtttatttgttgttaagttaaactggagaaagtttgtcatcctcattttcaaactgaaaactaatcaaatatagtgcctatttagtctcaaaataaggtaactattaacttgattatactatataatattctcaattacatttgaatttaaaaatattgagctcttgattacaatttaatacattgtaaaaagtattaaatcctttgaaacatcttttgttgcttatttagtttttgtttctacaggtcaaacatgattgctttctataaaagaaatgcttgagaggttgactataatggatatgtcacaggtataaaacagttgttttctaaaaacatgcatttagtatggcattctcttttagcaactgaattcccaacgagttttattaagctggatatcgaaatgaaggagctgccttaagcactttagaaaaagaatttttttacaattcattttgactctcatggctgaccatgtcattatgtctttaaattttggtaaatatgtagataccaagcattaataactaatgcacacagaaatttaatatacagcaattctttgaatgttccaggtgtacgtaaactaactgaaagtattaaggacatgcctgtctatacatgggtttcattgatggtatctgtatcatcttgacaaatcgtgaactgctgctgtatggctagactttgcctatttactctgttatgcaaacagtaatttttccctatgttatgaagagagacatattggcttgctttaatttacttatttatgaaattaaagcatgaataatatgtataatttgaattttttgtgactgatccttggcagtataaatgataaaagtaaatgtaatggaatcttttaattaggctaagatatgctatttcataacttatgtagaatgatttttatctatatactttgtccataaaattataattgtttatgtaattttattgtttcttatggaaacaattggaaaagtatatggaaaatgattatttcaaagaatatttatttaaagagggaagtgtagacttcttactgtaaaatatgtgattccaggcttaagaaattgattatattttaaaataattatttttttaaaaacgtaatttgtttttaaaagatgagtctccattcattggctaatccatacagcaaatatttgagtgtttgtgatatggcagtaaaaatgtgattactttgtatgtacattaaccaaaaccagtgaagtttgatggactgtgcatagagttttgcagcttttgagtagtgtgacagagtttgcctcttaaaattgttttgctaataagtcagaagtttaaaatgtgttatagtttgctaaaaaaaaatcaaattaactgcatataaaatggttcacttttatatagtcacatgtaatgggcctgaaaaagtttcttctttgattatgtagttactctagatacattcttttagggaagtgtatggtcaacatatatttactcagtatacagataaccacaaagttgttatttttaaccaaaatatacatttcataatgttggcactggagtattataagagatcatgaatgtttccttaattatcatggcaagattacctcacgttcagtatagtttagttttgtgtgtatcttacagtatgcatgttctgaaattatttgtgatcctgatatgtcacatataatagctttgttacctggagtatttgattaacctaaacagtttaagcattttgaattagttggagtttaaatggattacatttggtgtatattgtcttcattgaaaagatattgttggatatgccacatcagagttagcattgacttataaataaataccagaatttaccagagtacacttttctcttcagatgactcaattattaaataaaagaatatttcttatttctgggtcaatataaggtactgacttctgatgcataatcacttaagctatgtgagtttaaactggtatcttttcttagtggtacccattcaatgtaagctggtccatgggaatggacatgaagaggatttcacagtatgtagagcagaaggcacgtgaatgtgtttgctttggcttggagcttattaagttttgactacggttaaaataagtcaaatagtaagtggtaaaacacatttttgttagtattggaactttctggagaacataagggctatgagaatgcatatatatattttttaacatttcctatatatctaaggtaccaaagcactgagtctaatttacctattaagggagactctttaaaatcaactttataactaattcatactataagacagataatagctaaagttttggaataatttatattaaaagccgcaagtcttaaaaatccctggatatgacataaaaaggattttggcttcttttttgaagtatttaaaattaatcaccttagctctaccatatactagatttgtgaccgctacacaaattgtttatcatctttgggtctctattgccttctttataaaataagtgtaagttgttcagcctgcctcacagggctgttgtgaggaaataaaatgaaatggagtatgtgaaattgcttcagcaacagcaaagtgctacgtaaatgtaaagtgttgtttttagctaataatggatttaagtgtttggataattgtagatgcatttactttgataaagcgtgtgcttaaagtggtatcaccagtgatttctaacatgattttaaaaaaataaaaccccaattaaaatgttctttaatattcatttaatttgtgcatgacttgtggcctttttgtattttctcaagcctattactctagagctgtaaaagctcttgcacagcattgttgtgtcagtgtagaatagtggcataaataaatgaattaagctacatttccatgcaggcatttgcactttgaagttagggctgcccagtgccacatgcaaagagtgtatttggtctaaacagttctttccaaacaaccaaatggctgggcagcttgttgtcacggataaatgatataaaatgtaaccactgaacatttgacaactttgttgcattatcatttttaaaaaaagatgaagcatttcaaaatcttgttaacctggttatctcttggtatctctcctgacatatttgttttgctttaaattggattaaatggtttacaggttatctgaatctacagatttagtatgtctattatctggacatgattttgctatgcagttgtgataataaaaattctaattcctcaggtttggccttttaagttatggctgaagacctttaatgaactacttatgatgcattcagtgccatacaatagtgttttaagaagcacatggcctcattttccttagaaacaagacaaagcctttttaaaatgtttttttttcactttaaaatagggtattcaaagtggagtaacgtgtattttgaaatgattttgtgttctatatagaatgtcccagttaagattttacagaagcacctggaatatctcattaaaaatttaaaaactcttttcctgctctcttttgcttcattgtttgattttattaacttttatttaagtataaatacaatatgctgttggggatgagaatataaaaaaagtcatagttcctttgcctaaaaagcttaacattttagagcactactgttcaacagaattttatgcaattatgaaaagttatttgtgcagtccaatacagtagtgactggccataggcagctactgagcactttatatgtggctacatagagttgcatattgctaatagccactgttttgaacagtgtacctacagatggaaaatgaaacatgctatgttagtaactataatattacttatgaatttggtttctttggatcttgttacatgttgggttacattttggtagatggtaactaagagtcagaatcagaacctaaacatttttaaaattcttgctctaacttgaaaacagtttaaaagaaaaaaaatcagtgagactggagcacctgtaactaagaagttatgtaagaagaatgaaaggagactggatagtcttgagtcacaggaagaagaatggacaaagattgataaaccactatagaagatggagagtgaatgggtgcagcatttctggagaacaattttagcaatattaagatttttaaatgcacatgctccttaatttcctttataagtatttctcttacatatatactcacaaaaaagccaatgttccttgcagcattaccatagctaatagtagcaacctaattattaattgaagacctacaaatttggatggacttggaggtaaattccttttccttttttggtagcaaggcacagaactggttcaaaaggcccaagttgcctcaacaaaagaatgtgataacagaattttgaaggctccccttttctaacttgctgcaccagcaaactaccatataagtagtggtctagatattatatattctgcacattcccctccccaataaatgttatatagaccattatgacaattggcttaattagagccttttccttggtataccagttcatttgtgcctggctgggagttctgtggcataagagctcaggatattatgtgcactctacttttctactaaaccccattttacacttacactgcatggtgtatttgtatttatttatttttgcacaaggtcggcacaagagcagatggttagattttggtatttccatgtgatcctacacagctgttaaaggatatgctgttaatggaagtgtattcatgatattaaacaaaaaagtcatccagcaatatatacagtacgatacaacgggtgtgtgcatgcatgtatacttgggtaagaggggaccctgacctgatcaccacacagtcttgctgtgcttctcttcatgggatgaaaaattgaggagccaagggattatgcctacttggaatgcatgtttcattacccacttatatactatattattgaaacagtctttcgttgtctgagataacacctggagttcttgtccacttatatactacattattgaaacagtctttcgttgtctgagataacacctggagttcttgtcccacctccaagacgattatggagcacggacacaaaggtgaggttagagtgaaagtttaataaggtgaaagaagaaagctctctgccagcagagagggggtcccgaacgggagtgcccatcatgaggctggggtccaggtttttatggacggaaggggaaggaatgtgcttagtctgggggctgtcttggcgaatgcgtgactcggcttggcccgggaccagtcaggaggtgaaatgattcatagatgctgcttagcttggcccaggacctatcagaagctgaagtgaagtgtggccgaggaccaatcgggctgaggtgatgatacacagcagctggacttacagtcctaacaaaggaaagtagagcgcccatagaaacttacgagagcccactgtgcccatgcctacaaaaggggaataaacttttcctgggaacctgctgacaatacaaaggaccaaggcatttctatgccaggccttgttcccttatctgagtgagctggaggtttgtgcaagtttttatccaaatgggccgtaggtttttccatctgtgcagtcatgggcatgtctccaggcacaacaccctgtgctagttcccttattggtgcctgcagcttttttcccaggctgctttttatattatctggggataaggcactgactcatgagccaggggctctccaggacccttctcttgttacctacctaaggtaagctaactaaccggatccccacactcttgctgtgcctctcttcatgggatgaaaaattgaggagccaagggactatgcctacttggaatccatgttcctttacccacagaattctatactatgttatcagccagaaccccaggattccttgcctcatcagcctgaagcttgcttccaggatatgtgcaggccttttgtccaaatccatcctgaaaaaagactactacagatgtatatacccctatggctggcagtttgtgggaagtacagatgaagcttggatgtgcagactgagttgtccacatgcatgcatgataggcccctgtggcaggcttaagctagaagtaaaaagagacccaggggatcagggaagggcaggccaacctagtatcactttctagtacacttctgaagaatctgcgaatcgcatatttgaacctagatttctgttccttgagaatacatgttaaagtagaagagtataacattttatttgttggttaacgctcagctatttagacactgaaaatatgtcagggttggctttcatttgtattcttggcccagaccctacaaatgttaggagtcggccaggatccttacatgtgtgcacagctgagtggtttatagaacatgaatatttacttgtaagagaggctgtttttatgcatccttgtacccactctttcagctgtatttgctatccagattaaagcatactgacttgacgtttgccatgagctgagggctcacatttgacctttcagtatgcttgataagtaacactgccaccagtttagttgtatatttaccttcagttatgtttgttcccaaacctgcttatgtaggtggtagtcactgttgtagtcatgtaagtatgtaaaccaattatataaatatataaaccaaaataaatatgaaatgagtatgaaaaggtacttataagaaaagtacgagaaccattagagatgaagagtttaaaaagttgcaaagttagttgtggccaaagtaattgtgagtgataggggaagatttttaaaaataaattccaggactccaaatttatattccttcacttgtatctttaagttcctggtccattttacagaaacagaaactacaaatgatggatgatgcattatgtctatggttttgtaagaaaaacagtgagatactctaatcagctggtccatgcttaaaatgaacttagttcaaaacagaagattggccattgtaaccctctactgaaactgcctttttgagaaggtttattcagaactagatttgttatacacttggaaagtatttatttctaagaacctgataatttttcccttttcctgttacttttaattataatttccaaatatacagaaaagtagaaagccagtgctttgtgctcatcacctaatcaattgttaacattttgccatgtttgtgctatctattttgttttaaaatgtcacctgtaagtatgctatatgcatccatgatggcttttaaaaacagccacattctgttaacattcttagcaaaattaacagtaattctgtactattatctaatggatcagtccatactaaaatttcagttgtctcagaagtatctttttacagttatcttgttcaaatcaagatctagacagggtccacacattgtactccgttacatctcttaaatatttgattttacaatagttccctctgcttttaaatgccatttatgaaaaaaactgaggaatttgtctggtagaatgtcccgttttctgaatttagttgcttctctatatcctgtattagatctagagtttgagtaaatgcaggttcaatttttaggcaagaatccttcacaggtgtggctgtgtactttctatcacatcaggaagtacataatatatgcttgtcccaaatttagtgagattaagatcagtgggtttaggtgatgccagtctattataaagttccccatcaacctttcaccttaattttatcatctattgatgttgccctttcgattattttattaggagttacaaaatcgtgattgttttatcatcctccatttattagctggaactcttataagtactttggttacactaaaattcaattcatacaagaaagacaggataaatgcttgatgttttcccttatcaagttttagaatatttaatcttcaacttggcaatcttcaatcacgactgaattttattttttaaggagtcattataaactcaagaatttttatatttgatgtgtttcaatcaatagcaagtatgtgatgctcaagttttcccatgtcccatcacgttagcacctgtgttaatgatgccattaagctttgataacttacttcctcttggtgtaaccttccacttttttttattaacctactgagtacctacccgttctgagtgcattggatgagaggacttcaacagtaagcttgtatgtgcataggaaatttctggaaggaaaaacaaaaagttggtaaatgtcataacctgtaggaagtgaggaagattttttcttccttttctttctgtactgatagaattaaaaacaaagcttagaaaacaaatatatgatgggagtattttccgttttgtagaaataaattataattacagtaactggtttagtgaattatggttttcaaaaatttataagaagattaatatctgagccttaacaaccaccttttggattacaccgttaaaagaaccaaagtgagaggatcgcttgaggccaagagttcgagaccagcctgggcaagatggtgaggacgccctcccccccacccccgccacaccccgccctgctagcccccaacgtctctacaaaaaaagaaaagaaaaaagttaatcaggtacaaaattgtatccagccttaaactggagggcaacaggtcgctaaatcttgaatgtcataaaggcacctcaacttcatgaggaatagtgaacgcagctgctattttccactctatcccctagctctactaattgtatccaaaccaaacttcagggagttatgctgaatccctctagcaaagcacacgcactaaaaaaaccactcgtttatcagaagttcacatttaacgggcttggaaaacggctcagctgctgcctccagttcatcttccgctgtcgaaagcgtttcagaacttaaactctcagattgcctcagtgcgctgctgtagttgtcaattaggcaagagataaaaaagggctttggctaagtggctagattataaaagcgaggaatcgccagggctcagtgaacttctggcggtgaggatgcgacaagagtcacaggaaagccgaggctggggctggaccgtgggaacgtcccagcaggaaccaagccagcctccgccgctcagcacttgacggcggcttttgcggcggttgctgtgagtgccgtaaagcggagcggctgcagcctgctgttgagtgaggtaaggtacgggaggctcaggtcggtacccggggatgggtgggcgccttcagacaggtaccgctggcgactcgggtgcccttaccgggcatcctccagcattctgggcacctgcctaccccttggtgaggaggccggccacaggctgagcgcgctccgggctgggtactcctcagtcagtccacgagcatcgcgtggtagacttccacttggccagtccttcccgcacttctgggcgtgtcatcaggtgaaatcttaatcctgggacagatgaaaggttggaggacgatcgagactcttgtagtagccgggttagggtagtgacccctgacctcaggttatccgcccgcgttggcctctcaaagtgctgagattacagccgtgagccaccgcgcccggcctgaaatttacaatttctcatttaacatgaggtaagccacatttctcttggcttcagttttgtcagatgtggaaaaaaaaaaaaaaggacctagatgatatatcagattctttatgcttttgaagatagcacgtttccagtcagtaaaaatcaagctgtgaacaaatgacaaagtgaatgatagagcagtatattagaaattgggcagatggaagcccagtagaaaaggctgtgtttgagctagactctgaggataaatagggtttgaacgattggaaaccatctctgttgggccatggacaaagatatcaaatgcaggaataagcatttatattttagcgattctatttgtggacataagtttagtgagggtagaggatttgggaaggctggcattgaacggtgaaagaactcttagtggaaaggaagtgcagggtgttctgacaaggaagaagaaaggaaccggggaaatgccgaaagaacaatacgcaggacttgatttcttggatctgggtgatgatatttttaacctgcgtttctaaaaagtaagtttaagtgctgttggcaaaaatgggaattctgttgaattccagcatgcaatagtgtactgggaataaagtgatttagatcgtagagtgctgaggttgccaataactagcctcttggctgtcatttaattcttctagagcctattctccataaggtgatgttgggccagctgatctctcttctctaaagcctgtaaaactagagactgtgaggatggagagctagttactttcttctggactgggagaggacgatagttgacagagaataaaattgttaattttggggctggacgcggtggctcacgcctgtaatcccagcactttgggaggctgaggcgggtggatcacctgaggccaaggagttcgaaaccagcctggccaacatggtgaaaccctatctctactaaaaatacaacaaattagccgggtgtggtggcgggcgcctgtaatcccagctactcctgaggctgaggcaggagaatcgcttgaacttgggaggcagaggttgcagtgagccaagatcaggccactgcactccggcctgggcaacaagagcgaaactctgtctcaaaaaaaaaaaaaagttaattttgaacatgttaaatttgaggtgaggtgcaggaaatagagttgaaaatataggcagatagagtgcatggactgtaatttaaatagtgttttctctcacaggtggtagttaaaatcttgagaatggatttgctttcagggagagattgtagagagagtaactataggccatacccacagagaggaggttggagaaattattgaaggaggcatgtggatctcagagctaagagcaaggaaggagttctttttaaaaaagttacatatagttgtagattctcaggggcccagtgttgttattaagctaatttaacagcatttacagcaaataataagcacctacttctgggaattctggcagaaaataaataattcaaatagatataatctccactgcctaattgtctacccagaagtggtatcatttacatatttatttattcaacaaatatttatatgtttcaagcactgctggttctagggatataacgacgagcaaggtagacattgttcttatcctccctgcatgtaaagcccttagcatctacatcagtgcttttcaaattttaatgtacatatgaatcatctgaggattttattaaaatgtagattatgaatcagtaggtgggggctgaaaattctgtattactaacaagctccaatgtgatactgatgttcttaggaccatacttttaagtgacaagaatctagatcctgtttagcaaatatggccgttattaagccactaccactacccatcatctgtttctcctaggataaaataattttacttcttatgaaaataatatatgcttatacaaatattggaacaatatagaaaagtgtaaagaaccatgtaaaaatcactcctaattctccctacccagagataaccattattaatatttttgggaacattcatccagattttacatatgtacatacattcacaatttaagtgttgcactaagtacatgtcacactctaagccctgtgtttgattctatttgctgtatgattttattaagataaatacccaagtgtccagaaccaagcaattaagtacttgcattcttgagggagccacttaaaaataatttgggggccaggcacggtggctcacgtctgtaatctcagcactttgggaggccaaggtggatggatcacgaggtcaagagatcaagaccatcctggccagcctgatgaaaccctgtctctactgaaaatacaaaaattagctaggcttggtggcacatgcctgtagtcccagctactcgggaggctgaggtaggagaatcacttgaacctgggagcggaggttgcagtgagctgagattgtgccactgcactccagcctggcaacagagcaagaatccgtctcaaaaaacaaaaaaaaaaacaaaacaaaaaacaaactttgggagccggacagtgtctcatgcctataatcattccaggtgcccaagaggctgaggtgggaggattgcttgtgcctagcagtttgaggcagcagtgagctatgattgtgacactgcactccagcctgggtgacagagcaagactccatttcttaaaaaaataaaaacttgtgttacttcaaaaatggggagacattaacataattacatgtgggctctagtaaatgaatatttgtcatttcatttaggatgagaggagaatttttaaagttttaaaaaaaacttagtttttttcttactacaaaatcaattgatgttcacgtaagataaataaggaaaaaaaataaaagcacctacactcctcccaacccaaagacaatccttgctgtcttcaccttccttcctgctaacctgtcttatctatatctttcatttcagccactatctttccaaaaccctcttacaccatagtcattcagaaaggagtaactatgtatttatgatttttctggagcatctactggagaaactaaatttcattagctttttatcttcaagtaacagcatgtgtaggtagaagttatattgcaaaggattaagtgcatgaatggtaagcaggtaaagaaacttcttaaccctttgcagtctaatgtttacttccaagctgctgacagttgtgaaaagttagcagtcaaaggaaaagaaatggacaataagaaagaccaacagtatttagggaagatttgatagtagctgttgctactgggatatttttggcttttgagaacagctgaaaaatgtcgatttttttttttttttggtctgacctctgaattcattttcagacgcattttctctttatgcctgccaatctgctacatcatctctctaactataccttttcctaattacactactctctttcctctgtagttcagcctcctgttttattttgttcagagcatatttgaatgtcagttctgttttaatgaattgcctgaaggattcttcctgtgcgctgcacaaacgaaaccagttcactgagaccgtgctactgcagtaaagaaacagcttacttaacaatgatgctggctgtgcaaaggagttattactcaaatcagtctcgccaaagacttggtggttagtttttcaaggatagtttttagtttggtggcaggggactagggaatgagggctgctggttggctggggatgtgatgataagggtgtgaaaaatggtccttgtgtgctgagtccacctctgggtggggagccacgtgactggttgggtcatgagtcactagttcacctctaggtagtgtcagttggtccagaatgcaaaggtctgaaaaatatctcaaaagaccaatcttaggttctgtagccagggaaaatataaatcctgtgtcctctggaaaaaagactggttatcatttaactacatgttaccagaattcaggtccctctcataatcctaatcttgtagtctttcattacctttataaaggcagtttagttttggaaaaggttactatcatccttgctttaggttaaactgtaaactaaattcctttcaaagttagcttggcctgcacccagaaatgaccaaggacagattggaggtcagaaacaagatggaatcaactatgagatttctcttagctgtcataattttgcaaaggcagtttcactctctgattcatactatctatgcctcactcttactccccaatatccccaaataagtcggggatcccacagcataaggatatggctaggctctcacatatcatcttatgaacctaagttaggtgtcagggaaggtttttgattccacttccccccactcctgccttctggatcatctctcttgatatatcattcattcattcattcattcaaacagacccctacctaggtgattctcaaaagagtggggtctggggctggaggaggtgtcagggtaaaccagttaccaaaagtctttcatactaataccttcaaaggacaaatgcaaatgtaaaaaggaagctgaaagaatatgcagtggggttccaagatggccgaataggaacagctccagtctacagctcccagcgtgagcgacgcagaagacgggtgatttctgcatttctaactgagatactgagttcatctcactggggattatcggacagtgggtgcaggacagtgggtgcagcgcaccgagcgtgagccgaagcagggcaaggcatcacctcacccgggaagtgcaaggggtcagggaattccctttcctagccaagggaaggggggacaaatggcacctggaaaatcgggtcactcccaccctaatactgtgcttttccgacagtcttagcaaacagcacaccaggagattatatcccacgcctggctcggagggtcctatgcccacggagcctcactcatttgtagcacagcagtctgagattgaactgcaacgtggcagcgaggctggggggggggcacccgccattgctgaggcttgagtagataaacagaggggccgggaagctcgaactgggtggagcccaccacagctcaaggaggcctgcctgcctctgtagacttcacctctgggggcagggcatagccaaacaaaaggcagcagaaacctctgcagacttaaatgttcctgtctgacagcttggaagagagtagtggttctcccagcatggagcttgagatctgagaacggacagactgcctcctcaagtgggtccctgaccctcaagtagcctaactgggaggcaccccacagtaggggcagactgacacctcacacagccgggtacccctctgagacgaaacttccagaggaacgatcaggcagcaacatttgctgttcagcaatattcgctgttctgcagcctctgctgatacccaggcaaacaggatctggagtggacctccagcaaactccaacagacctgcatctgagggtcctgactgttagaaggaaaactaacaaacagaaaggacatccacatcaaaacccatttgtacatcaccatcatcaaagaccaaaagtagataaaaccacaaagatggggaaaaaacagagcagaaaaactgaaaattctaaaaatcagagcacctctcctcctccaaaggaacgcagctcctcaccagcaatggaacaaagctggatggagaatgactttgacaagttgagagaagaaggcttcagacgatcaaacttctccgagctaaaggaggaagttcagacccaacacaaagaagttaaaaaccttgaaaaaagattagacgaatggctaactagaataaccaatgcagagaagtccttaaaggacctgatggagctgaaaaccatagcacgagaactacatgaagaatgcacaagcttcagtagccgatttgatcaactggaagaaagggtatcagtgatggaagatcaaatgaatgaaatgaagccagaagagaagtttagagaaaaaagaataaaccgaaatgaacaaagcctccaagaaatatgggactatgtgaaaagaccaaatctgcgtccgattggtgtacctgaaagtgacagggagaatggaaccaagttggaaagtactttgcaggatattatccaggagaacttccccaacctagcaaggcaggccaacattcaaattcaggaagtacagagaatgccacaaagatactcctcgagaagagcaactccaaaacacgtaattgtcagattcaccaaagttgaaatgaaggaaaaaatgttaagggcagccagagagaaaggtcgggttacccacaaagggaagcccatcagactaacagctgatctctcggcaggaactctacaagccagaagagagtgtgggccaatattcaacattcttaaagaaaagaatcttcaacccagaatttcatatccagccaaactaagcttcataagtgaaggagaaataaaatcctttacagacaagcaaatgctgagagattttgtcaccaccaggcctgccctaaaagagctcctgaagggagcactaaacatggaaaggaacagccgataccagcctctgcaaaaacatgccagattctaaagaccatggatgctaggcagaaactgcatcaactaacgaggaaaatcagcagctaacatcataatgacaggatcaaattcacacataacaatgttaaccttaaatgtaaatgggctaaatgccccaagtaaaagacacagactggcaaattggataaagagtcaagacccaccagtgtgctgtattcaggaaacccatctcacatgcaaagacacacataggctcaaaataaagggatggaggaagatctaccaagcaaatggaaaacaaaaaaaggtaggggttgcaatcctagtctctgataaaacagactttaaaccaacaaagatcaaaagagacaaagaaggccattacataatggtaaagggatcaattcaacaagaagagctaactgtcttaaatatatatgcacccaatacaggagcacccagattcataaagcaagtcctgtgtgacctacaaagagacttagactcccatacaataataatgggagactttaacaccctactgtcaacattagacagatcaacgagacagaaagttaacaaggatatccaggaattgaactcaactctgcagcaagtggacctaatagacatctatagaactctccaccccaaatcaacagaatatacattcttctcagcaccacaccacacttactccaaagttgaccacatatatggaagtaaagcactcctcagcaaatgcaaaagaacagaaattataacaaactgtctctcagaccacagtgcaatcaaactagaactcaggattaagaaactcactcaaaaccgctcaaatacatggaaactgaacaacctgctcctgaatgactactgggtacataacaaaatgaaggcagaaataaagatgtgctttgaaaccaaggagaacaaagacacaacataccagaatctctgggacatgtttaaagcaatgtgtagagggaaatttatagcactaaatgcccacaagagaaagcaggaaagatctaaaattgacaccctaacatcacaattaaaagaactagagaagcaagagcaaacacattcaaaagctaacagaaggcaagaaataactaagatcagagcagaactgcaggagatacagacacaaaaaacccttcaaaaaatcaatgaattcaggagctggttttttgaaaaggtcaacaaaattgatagaccactagcaagactaataaagaagaaaagagagaagaatgaaatagacgcaataaaaaacgataaaggggatatcaccaccgatcccaccgaaatacaaactaccatcagagaataaacacctctacacaaataaactagaaaatctagaagaaatggataaattccttgacacacacactctcccaagactaaaccaggaagaagttgattctctgaatagaccaataacaggctctgaaattgaggcaataattaatagcttaccaaccaaaaaaagtccaggaccagatggattcacagccgaattctaccagaggtacaaggaggagctggtaccattccttctgaaattattccaatcaacagaaaaagagggaatcctccctaactcattttatgaggccagcatcatcctgataccaaagcctggcagagacataacaaaaaaagagaattttagatcaatatccctgatgaacatcgatgcaaaaatcctcaataaaatactggcaaaccgagtccagaagcacatcaaaaagcttatccaccatgatcaagtgggcttcatccccaggatgcaaggctggttcaacatacataaatcagtaaatgtaatccaacatataaacagaaccaacaacaaaagccacataagattatctcaatagatgcagaaaaggcctttgacaaaattcaacaactcttcatgctaaaaagtctcaataaattaggtattgatgggacgtatctcaaaataataggagctgtttatgacaaacccacagccaatatcatactgaatgggcaaaaactggaagcattccctttgaaaactggcacaagacagggatgccctctctcaccactcctattcagcatggtgttggaggttctggccagggcaatcaggcaggagaaagaaataaaagatatttagttaggaaaagaggaagtcaaattgtccctgtttgcagatgacatgattgtatatctagaaaaccccattgtctcagcccaaaatctccttaagctgataagcaacttcagcaaagtctcaggatacaaaatcaatgtgcaaaaatcacaagcattcttatacaccaaataacagagagccaaatcatgagtgaactcccattcacaattgcttcaaagagaataaaatacctaggaatccaacttacaagggatgtgaaggacctctttaaggagaagtacaaaccactgctcaacgaaataaaagaggacacaaacaaatggaagaacattctatgctcatggataggaagaatcgatatcttgaaaatggccatactgcccaaggtaatttatagattcagtgccatccccatcaagctaccaatgactttcttcacagaattggaaaaaactactttagagttcatatggaagcaaaaaagagcccgccttgccaagtcaatcctaagctaaaagaacaaagctggaggcatcgcgctacctgacttcaaactatactacaaggctacagtaaccaaaacagcatggtactggtaccaaaacagagatatagaacaatggaacagaacggagccctcagaagtaataccacacatctacaactatctgatctttgacaaaactgataaaaacaagaaatggggaaaggattccctatttaacaaatggtgctgggaaaactggctagccatatgtagaaagctgaaactggatcccttccttacaccttatacaaaaattaattcaagatggattaaagacttaaatgttagacctaaaaccataaaaaccctagaagaaaaccaaggcaataccattcaggacataggcatgggcaaggacttcatgtctgaaacaccaaaagcaatggcaacaaaagacaaaattgacaaaagggagctaattaaactgaagagcttctgcatagcaaaagaaactaccatcagagtgaacaggcaacctacagaatgggagaaaatttttgcaatctactcatctgacaaagggctaatacccagaatctacaaagaactcaaacaaatttacaagaaaaaaacaaccccatcaacaagtgggcaaaggatatgaacagacacttctcaaaagaagacatttatgcagccaacagacacatgaaaaaatgctcatcatcactggccatcagagaaatgcaaatcaaaaccatgataagataccatctcacaccagttagaatggcgatcattaaaaagtcaggaaacaacaggtgctggagaggatgtggagaaataggaacactttcacactgttggtgggagagtaaactggttcaaccattgtggaagacagtgtggtgattcctctgggatctagaactagaaataccatttgacccagtgatcccattactgggtatatacccaaaggattataagtcatgctgctataaagacacatgcacatgtatgtttattgtggcactattcacaatagcaaagacctggaaccaacccagatgtccatcagtgatagaccggattaagaaaatgtagcacatatacaccatgaaatattatgcagccataaaaaaggatgagttcatgtcctttgtagggacatggatgaagctggaaaccatcattctcagcaaactatctcaaggacagaaaaccaaacatcgcatgttctcactcataggtgggaactgaacaatgagaacacttggtcacaggaagggggacatcacacaccggggcctgttgtgggatgggagcaagggggaggcgtagcattggtagatatacctaatgtaaatgatgagttaatgggtacagcacaccaacatggcacatgtatacatatgtaacaaacctgcatgttgtgcacatgtaccctagagcttaaaatataataataaaaaaaataagtaaataaaaaagaatatgcagtgctgctcttcactgtagaaagagcctgagaattatcttgaactccaaatcctgtaccttttttcatcacagttgtgtatgggttttatctactactagtttttttccaagccttttcacatcttgacacatagtaaatttgaccaagaaaagatgaaaggaaacataaaagaatgtgttcttggctggagatgacctactcttggggtctagctgccccaaagactgagaggattgttaactctgacacctataacccattcatgatttagttggtaagcagatctgcccatttctttcttcttcattgccagatctcagttcatgcactagttatgccctgcttccacttcatctaagaataattctgtgtcgcaatataccataattatatattaatcttctcatatttgcattagaactttaagattattgggctacttaaacttcgtaactcccctcgttacatcttttttttccctgaaaacatttgtcatttctctcccaaccactgcctcattttaatttactatctctgcaatactttttcttttcttttccattagagatgatatgctgtcttctttaggaaactttacctaagtgtaagtaaggaaatgaatgctatcctccctagtgtttttattatgatagctaaaatgtaacatataaaaagaagtgtatatagaaacaatatttttgttttagttctatgccatatctctctgtaggttattttttatatttttaaacgtttattttttgaaggttggaaccagatatgtgagtttaaggggctttaaactcttttaaaaatcttttttttttatatttcaaattctgttttattgtaaaagttcctgcagaacagaaaagttttatttaaatagttttctgttttcttgagcattgtgcagtgtatttttagtatacttagcatacttactattacttgatgttaattcagccaattttaggctggtggggaagatgattcatgtacactaacagttataatgcaaaatagaaactagtaaaagcctcaaggttagttgcctctccttgtgcttccatagtaacccgtgcttattccttcattgcaactatactgtattgttattgcctctatatttatctctgatagagtccatcataaactagaacagtggttcttaattgatgtgggggtggtaaggaatggggcttgcgcattttggaaaacatcttctcatattctttttcaggtacatcactctctccaccactatcactactgcccttcttcttttgaaaactcctgtactcacctttaagcccttcaaaattagggaagtgtatcttatttgtcattttatctctagtgcttagcatttttttttggcatctgtgcccattaaggtagacagtaactgtttatttgttgcaggaaggtaaaactaggttggaggtggagggagcacttctaacctggaagaatattgaagacttccttgaagaagtgtcatttgagaggagctatgaaaagaaagtaaactggttttatggaagtaaatgagaacattgcagacaagaggtaatgggcaaaaacacagaggcaggaaagtgtaggatgtattccaggaatactcatgcaaaaaccatagactatgtgaagtgtgagaaagcttatagtaaatttgcctgtattcagtcagattgtgaatacccctttataccattatatgtaatttgaactatttgtaggtggtagggaactattgaaaagttttgattgtggtgtaacttgatttatctgtcagcaacttgatacatctgtcagtgtataggtaagattgtggatacagagaaagtggagacagggacatcagttaaaattaggacattaggtacaattagagtttagaatgacagtgaagaaggaaggaattgatgcaagaggtattttaaaggtaaaatcaacatactatggcttctttttttcagtatcacattattcatttttaagtggttactgaatattcctaatgaagcggtagtgctagtgaaaaggaacattttgataggcgaatctttctcttttgtgactgaattgccttggcatttatagaaaataaataatgaagttaattggatatcatcttgataataaaaatgtaattaagtttttgatattatggtttggaggtttattttataagaattagttgtaaactagagaagaaagaacaagatattaatttagattttatgcctgtagtagcttatataggcaggcctattatgtgttctttcccatttattaatttgggcttagaagaagctgagttatggcctactctgagtgccactttagatttcactaggaatcagcatagaatacattaatgcactgtttaatacaagtacaagaacttgagttgaaatcttgaaaatgaagggcagtctccttgttaatcttgtgagctgccctcatcagagtataggttgagcatcccaaatctgaaaattcaaaatctgaaatgctccaaaatctgcaacttttgcgtgctaatatgatgctgaaaggaatgttcattggagcatttcagaattttggattagggatgttcaactggtaagtgtaatccaaatattctggaatcctaagaagtccaaaatacttttggtcccaagcattttggataagggatactaaacctctatttgataattgtatttccatgggttttaactgaatacaaaaactaataccatcatcaatgttgattgatattgttttcacagttttgggagatacaaaataattatgatttattaggttatcgttgcttaatatacattactgatcaggtgaattgttcacatcactattggtattatttctcttaagtagtttcttgagactgtatatatatatatatatattttagtgtttgctttatatagtcatcagctctggcagctcatttggattgttttaaaaccccaaaccaagacttgattttaagatggtaaagacatttgtgccctattctatctgaaattaccatgaaacaacaaggaaactgagagaaagagatgtaattacatctttgctgagactagaagacctgtaactccaaactgaaatatttgagaaatggcagccacatgtaagcaggaagaggttaaaagagaatgctggtagaaagagatctcagatagagctggcagagcaaagagtcctcttctgtttgcagtgggatcaggatgcatagaaaggcaatgggaatttccttggattgtttggcaacatgaactagcaagaaaggaagagtgaatgaggaagtgcacagataccccatctttgcaggaagcactctcttgctgaggcaaagtagaggagagatagtgagtggccctttgctgcctgtctctgacatctggaagaagtaatgtttaaatgcttttcccacttgttctcatacacattctctgcctttctcacatatacacatgtacaaaatactctgtcagaaagagttttcttgtataccagagactaccctctagtctagaatacacccttatttctttcttccatagttaaggcgtaaattatattcccatttagaaaagtaggtgaggactgggtgccgtggctcatgcctgtaatcccagcactttgggaggctgaggcaggtgggttgcttgaggtgaggagttcgtgaccagcctgaccaccacagaaaaaccccgtctaaactaaatatacaaaaattagccgagtgtggtggcaggcacctgtaatcccagttactcgggaggctgagataggagaattgcttgaacccaggaggtgaaggttgcagtgaactgagatcgtgccactgcactccatccagcctgagtgacagagggagactctgtctcaaaaaaaaaaaatgcttaattgcagttctgaaaatagagaattcaatgttataacagaaaaaatatttaagaaaaccttctgcaaagaaaagacatctttaggtcaggctcagtagtagctcacacctgtaattccagcactttgggaggctaaggcaggaggttctcttgaggctgggagtttaagaccagcttgggcaacatagcaagaccctgtctttacaaataaatttttaaaaaattagctgggcatggtggcacatacttttactcatggctactcaggaggctgagataggaagatcacttaagtgtgggagtttcgggttacaatgagctatgattgcaccattatacttcagcctggacgacaaagtgagaccctgtctcaaaaaaaaaaaaatctttattctacagattgaaaggaaacacactgaatgaggaaaaactaacatacggtcatcaacatccttgtataacctagtttttaaaaaaattggatttcaaaggtaaggaatgcattctttgctcatcccaataaaaagattaaactacctatcaggagttggtttgggaaatcagatattgtcaagggaatatttagcactacaggacaatggtacaaagtgtgtaagtcattggggaaagacagtgtaacctcaaagccaaattgacaactatttttgaacaaggcaaaagctcaaggtaagtggtacccctaagttctttttgataaactgcaagaagatgaatatcagtcatacagtagatgaacagagatgatatagcaaatggattggcagggaacattgtaggaataagaccaaaataactatgagatttgtagttatagaatacaatagaactgtaacatgtagaaataattaataaaagtcaagattgaaagaggagagaagacagaatgtagtataaatttgttggtttcttcttattttatagctggagaacaaaagacatataaaccttagatatcaagcataagagaggtgtcagtatatttgaaggattgaaggaataaatgtaagcatttgaagaactaaatgtgtttaaccaaaatcaaacagtggagacaaggtaggaagaagtagaactgtattaaatttcttatcctaaaggaataatcagagatgagacctaagatgaaagaacaaaatgtttattgtggcattctttacagttgaaaaaactgaaaacatacatggagtataaataaaaactgaccacatcctagatcacacacaaacttgaaaagcaacaaagagctgtcttacaggccatgttccttgactaaaaacggtctcagtttctcctttggaagtggttctcagcattgtcagcagcaccagcatcatttgggaacttgtcagaaatgaaaattctgaggtctcataccggatttactgaatcagaaactggaggagaaaagcacctctcaaccttgttggtcagtttttataaatatcctatttatgttttcagttatttacagttataaaaaaaagtgataataaacatttttgttttttcatcattggtctcatatttgattatttctttagcatagacaatgaccagatcaaagaatgcctgtggaaatttaattttttctttgttctattgttggttattacaggtacaaaattaaagaggtttttgtttctttaaaaatatcttttttgttcacagaaaacaaaattatcttcctttccaaatccaaaaagatgaaaacgactgagatactttcaaaagacaaccaagtgagcagcacagactaatgagtagaatcaataagaacgtggttttggcccttttaacgctgacaagttctgcatttctgctgtttcagttgtactactacaagcactatttatcaacaaaggtaattttattccttctttcttatcattcctcctttcttatcattgtatattttctgatcacacttctctttgcaatacataatattaatcatgggtattcaaattcttgcatctttgcgaggtgtggcaaacaattaaaaattcagttaaatatacttgtaatagcacactaaagacaggtgctaagtttcaaggatgtttaatctattggaatttcctgagctagttatttaaaaattattattttgttaaacagattatccttcatttaaatgaactcaatgataaataattttgataaaatgtcaaaattagtttattttagtacagcatatattttaatttagtacctactggggaagtataatggtatgacttacctttatctgtatgtataggaataaagtagagacaatgatgtggaaatcaatagcttctgaagattccgtagaatataccagataaggaattccaaagttgagatggtgttgttacattgtgaaaagttgccaaacactccctctggggtgtattataataattactaccatcactgataattgtactagatgctttccatgctcagtttagtcctaaaaacaatcatggggaagaaaaaaaattttttttgtttttatgtttttatcctcatgtcttaattagaactattcatcagaattaatcactttgcgcccctcctcaactagaatggagtatacttccctgccttttttatgttgggcttgaccagtagaatgttaacagacatgtgcagaagctttgaataggctgttgtgatttgacttagtttttatgctcccctgacctataggagaagagaaaaatgtatggagcagaccaaagcatagctgcccagctgactcacagatttgtgagggaggaaatagatgcttataagccataagactgggggaagtttattatgcagcattgttacatggagttattagacctaattttgacagataagaaaactgaaacttttctttttttttttttttaattaatttattttttttattatactttaagttttagggtacatttgcacattgtgcaggttagttacatatgtatacatttgccgtgctggtgtgctgcacccactaactcgtcatctagcattaggtatatctcccaatgctatccctccccactcccaccaccccacaacagtccccagagtgtgatattccccttcctgtgtccatgtgatctcattgttcatttcccacctatgagtgagaatatgcggtgtttggttttttgttcttacgatagtttactgagaatgatgatttccaatttcatccatgtccctacaaaggacgtgaactcatcattttttatggctgcatagtattccatggtgtatatgtgccacattttcttaatccagtctatcattgttggacatttgggttggttccaagtctttgctattgtgaataatgccgcaataaacatacgtgtgcatgtgtctttatagcagcatgatttatagtcatttgggtatatacccagtaatgggatggctgggtcaaatggtatttctagttctagatccctgaggaatcgccacactgacttccacaatggttgaactagtttacagtcccaccaacagtgtaaaagtgttcctgtttctccacatcctctccagcacctgttgtttcctgactttttaatgattgccattctaactggtgtgagatggtatctcattgtggttttgatttgcatttctctgatggccagtgatgatgagcattttttcatgtgtcttttggctgcataaatgtcttcttttgagaagtgtctgttcatgtccttcgcccactttttgatggggttgtttgtttttttcttgtaaatttgtttgagttcattgtagattctggatattagccctttgtcagatgagtaggttgcaaaaattttctcccattttgtaggttgcctgttcactctgatggtagtttcttttgctgtgcagaagctctttattttaattagatcccatttgtcaattttgtcttttgttgctattgcttttggtgttttggacatgaagtccttgcccatgcctatgtcctgaatggtaatgcctaggttttcttctagggtttttatggttttaggtctaacgtttaaatctttaatccatcttgaattgatttttgtataaggtgtaaggaagggatccagtttcagctttctacatatggctagccagttttcccagcaccatttattaaatagggaatcctttccccatttcttgtttttctcaggtttgtcaaagatcagatagttgtaggtatgcggcattatttctgagggctctgttctgttccattgatctatatctctgttttggtaccagtaccatgctgttttggttactgtagccttgtagtatagtttgaagtcaggtagcgtgatgcctccagctttgttcttttggcttaggattgacttggcgatgcgggctcttttttggttccctatgaactttaaagtagttttttcgaattctgtgaagaaagtcattggtagcttgatggggatggcattgaatctgtaaattaccttgggcagtatggccattttcacaatattgattcttcctacccatgagcatggaatgttcttccatttgtttgtatcctcttttatttccttgagcagtggtttgtagttctccttgaagaggtccttcacatcccttgtaagttggattcctaggtattttattctctttgaagcaattatgaatgggagttcacttatgatttggctctctgtttgtgtgttgttggtgtataagaatgcttgtgatttttgcacattgattttgtatcttgagactttgctgaagttgcttatcagcttaaggagattttaggctgagacaatggggttttctagatatacaatcatgtcgtctgcaaacagggacagtttgacttcctcttttcctaattgaataccctttatttccttctcctgcctaattgccctggccagaacttccaacactatgttgaataggagtggtgagagaggacatccctgtcttgtgccagttttcaaagggaatgcttccagtttttgcccattcagtatgatattggctgtgggtttgtcatagatagctcttatcattttgaaatacgtcccatcaatacctaatttattgagagtttttagcatgaagggttgttgaattttgtcaaaggctttttctgcatctattgagataatcatgtggtttttgtctttggctctgtttatatgctggattacatttattgatttgcgtatattgaaccagccttgcatcccagggatgaagcccacttgatcatggtggataagctttttgatgtgctgctggattcggtttgccagtattttattgaggatttttgcatcaatgttcatcaagaatattggtctaaaattctctttttttgttgagtctctgcccggctttggtatcagaatgatgctggcctcataaaatgagttagggaggattccctctttttctattgattggaatagtttcagaaggaatggtaccagctcctccttgtacctctggtagaattcggctgtgaatccatctggtcctggactttttttggttggtaagctattaattattgcctcaatatcagagcctgttattggtctattcagagattcaacttcttcctggtttagtcttgggagagtgtatgtgtcaaggaatttatccatttcttctagattttctagtttatttgtgtagaggtgtttattctctgatggtagtttgtatttcagtgggatcggtggtgatatcccctttatcgttttttattgtgtctatttcattcttctctcttttcttctttattagtcttgctagtggtctatcaattttgttgaccttttcaaaaaaccagctcctggattcattgattttttgaagggttttttgtgtctgtatctcctgcagttctgctctgatcttagttatttcttgccttctgttagcttttgaatgtgtttgctcttgcttctctagttctcttaattgtgatgttagggtgtcaattttagatctttcctgctttctcttgtgggcatttagtgctataaatttccctctacacattgctttaaacatgtcccagagattctggtatgtcgtgtctttgttctcgttggtttcaaagaacatctttatttctgccttcatttcgttatgtacccagtagtcattcaggagcaggttgttcagtttccatgtagttgagcggctttgagtgagtttcttaatcctgagttctagtttgattgcactgtggtctgagagatagtttgttataatttgtgttcttttacatttgctgaggagagctttacttccaagtatgtggtcaattttggaataggtgtggtgtggtgctgaaaaaaatgtatattctgttgatttggggtggagagttctgtagatgtctattaggtccgcttggtgcagagctgagttcaattcctgggtatccttgttgactttctgtctcgttgatctgtctaatgttgacagtggggtgttaaagtctcccattattaatgtgtgggagtctaagtctctttgtaggtcacataggacttgctttatgaatctgggtgctcctgtattgggtgcatatatatttaggctagttagctcttcttgttgaattgatccctttaccattatgtaatggccttctttgtctcttttgatctttgttggtttaaagtctgttttatcagaaactaggattgcaacccctgcctttttttgttttccatttgcttggtagatcttcctccatccttttattttgagcctatgtgtgtctctgcacgtgagatgggtttcctgaatacagcatactggtgggtcttgactctttatccaatttgccagtctgtgtcttttaattggagaatttagtccatttacatttaaagttaatattgttatgtgtgaatttgatcctgtcattatgatgttagctgctgattttcctcgttagttgacgcagtttcttcctagtctcgacggtctttacattttggcatgattttgcagcagctggtaccggttgttcctttccatgtttagtgcttccttcaggagctcttttagggcaggcctggtggtgacaaaatctctcagcatttgcttgtctgtaaagtatttaatttctccttcacttatgaagcttagtttggctggatatgaaattctgggttgaaaattcttttctttaagaatgttgaatattggcccccactctcttctggcttgtagggtttctgccaagagatccgctgttggtctgatgggcttccctttgagggtaacccgacctttctctctggctgcccttaacattttttccttcatttcaactttggtgaatctgacaattatgtgtcttggagttgctcttctcgaggagtatctttgtggcgttctctgtatttcctgaatctgaacgttggcctgccttgctagattggggaagttctcctggataatatcctgcagagtgttttccaacttggttccattctccccatcactttcaggtacaccaatcagacgtagatttggtcttttcacatagtcccatatttcttggaggctttgctcatttctttttattcttttttctctaaacttcccttctcgcttcatttcattcatttcatcttccattgctgataccctttcttccagttgatcgcatcggctcctgaggcttctgcattcttcacgtagttctcgagccttggttttcagctccatcagctcctttaagtacttctctgtattggttattctagttatacattcttctcaatttttttcaaagtttttaacttctttgcctttggtttgaatgtcctcccgtagctcagagtaatttgatcttctgaagccttcttctctcagctcatcaaagtcattctccatccagctttgttccgttgctggtgaggaactgcgttcctttgtaggaggagaggcactctgcgttttagagtttccagtttttctgttctgttttttccccatctttgtggttttatctacttttggtctttgatgatggtgatgtacagatgggttttcggtgtggatgtcctttctgtttgttagttttccttctaacagacaggaccctcagctgcaggtctgttggagtaccctgccttgtgaggtgtcagtgtgcccctgctgcggggtgcctcccagttaggctgctcgggggtcaggggtcagggacccacttgaggaggcagtctgccggttctcagatctccagctgcgtgctgggagaaccactgctctcttcaaagctgtcagacagggacattgaagtctgcagaggttactgctgtctttttgtttgtctgtgccctgcccccagaggtggagcctacagaggcaggcaggcctccttgaactgtggtgggctccatgcagttcgagcttcccggctgctttgtttacctaagcaagcctgggcaatggcgggcgcccctcccccagcctcgctgccgccttgcagtttgatctcagactgctgggctagcaatcagcgagattccgtgggcgtaggaccctccgagccaggtgtgggatatagtctcgtggtgcactgttttttaagccggtctgaaaagcgcaatattcgggtgggagtgacccgattttccaggtgtgtccgtcacccctttctttgactcagaaagggaactccctgacaccttgcgcttcccaggtgaggcaatgcctcgccctgcttcggctcgcgcacggtgcgcgcacccactagcctgcgcccactgtctggcactccctagtgagatgaacccggtacctcagatggaaatgcagaaatcacccgtcttctgcgtcgctcatgctgggagctgtagaccggagctgttcctattcggccatcttggctcctacccgaaacttttctttttttaagagaggatctcgcttcgtcacccaggctgaagtacagtggcataatcatagctcactgtaaccttgaactctggggctcaagcagtactcctgcctcaatctcctgagttgttaggaggactacaggcacatgccatcacgcctgactaattaaaaaaaattttttgtagagacggggtctcgctgtgttgcccaggctggtcttgaactcctggcctcaggcagttctgtcacctcaggctcccaaagtgctgggattacaagtatgggctactgcaactggcctggaaaaccaaaattgttaacagagatgtgaaataatttacccatacaaaccacccaatatctaatgtgtatagctgacctctaatgtccctagctccattttttccaggctatataattttaaaaataacagactatactgattctacttttgatcttggctgtttatccaatgaatgtctttctgtgacatcttcaaccctttcctcattattttcttaggataaagtcctagagtagaaattctagatctaatatgcacattttagatttttgttatatattacaaagttatccttcataaggataagcagtatacctgatttctcatatcttttcataaataggaataacaataataatggcatctgtttcagttagagatggctggctaatagtagcttaaacaaatagaggaattatctgtccatatctataagtctagagcctctaaaattctcttggtatttcctgtgttacagtcaaggctagaaggaataatagtgtgatctagcaggcttctagttttgtgacagtggccagcagattcccaaatataagagaatctggggaagtaaggttttactattgttatttagcttttctagcctctataatagagattgcaaaagagaaggggtttgggaatgggtgtcaggtcagcttacctatagtgcctgccatagcagctaacattttttgatgtgcttgattgagcaggccctatgcgaagcactttaccaacatttaattcttaaaacaagttgagtagatcttgttcttcctgtttttccagcaaaaacattgaggttttgagagacttactaattttcccaatatcacatagttattaagtgggggagatgaacctgaggagtctaccccaaaacctcattcattaatttttagtgttcgtaatattcagaaactgaaagctattcaactccattagaggtcgtttctttgattactagtggggttaaacatctttccatatgtatattggttctttttagttgtattcttacttcttcttatttgtgtctttcatatatgttcctgatgatgttgtctttttctgtagctgttctttatagtttgaagaatattaaaccttcatcatatatatttcaaatatttttcctgacttgtaatttgccttttaactttatattcatgatgtactccctcaataaattagtacttaatgtataaatagacagatgtcaaaatctgttttccttagggcatctgttttttatgttataagtagcccaagattatgggaatatttaactgtatttttgtctatttaatgtttaaattttttcactaaaatgaatttattttagtatgaggtatgaattagacatctaacttacatttttccacaatgattaaccaattgtcccaatatcccttattgaattacccattactttaaaaatcccatcttaattatatattaaattctaataaagaactgctgtctcaacccttttcccttggtggcagtgtaacatagttgttgagagcatgaacatcagtttgagattaaacctcatctatactgcttattagctgtgggatcttgagttaattacttgacttctaaatgcctttgtttccttatctacaaaatgggaggcaataacagtaccacctcatagacttgtgaagcttaaatgaattgatatacataaactatttggaacaatgcatgttatacagaaagaaaccagtaaaaattggctattattattattttttaattttataatgaaaaatagtatttgttgtattgtgtccataccatacaaactgccttagtaataatgccttattcattaaagaaaatataatctttgaacagaagtggtatgtaattaaagttcaggtaacctttatataccattaattttgtaaagttcattattcatactagattcttgttttttatgtttacttttgataataggtagacattataacatctaagttctaaaatatcacagattatttttattttattgaaatatatggagtgggtgcagtggctcacacctgtagtcccagaatttggggacactgaggtgtgcagattgcttgagcccaagagtttgaaaccagccatggcaccatggcaaaaccccatttctacaaaaaatacaaatattagcccagcatggtggcgtgtgcctgtagtcccagctattcaagaggctgaggtgagaggatcacttgagcttgggagattcaaggctgcagtgagctgtcattgcgccactgcactccagcctgggtgacggggagatcgtgtcttaaaattttttttttttaacatatggaaattatattaaaccgtttgtagcccagtaattgtatcctttaaaatggaatttttaaatttactcatgagttcagaaactgttatttaaaagtcacaatttgtagagtattttgccaaggcaatagaaacaatgaggtggtttcttcctgcccaatatttataatttaatttgggacagatgctgatgagagtatagatgcttcctgtatgttatagtgtgaaaacaggatactgtctgtaaggaatacaagcagtttctctatgccagtaggaaaaaaaaatgctttatttaaaaatagtaaggagaccaggtgcctgcctgtaatcccagcactttgggaggcttaggcgagaggatcgcttgagcccaggaattcaagaccagcctgggcaacatagtaagatctcatctctgctaaaaataagaaaattagctggttgtggtggtgcacgcctgtagtcctagctacttgggacactgaggtgagagaatccctctgagcccaggagtttgagtttacagtgagctaagatctgcactccaggatggacaagagagggagaccctgtctcaaaaaataaataaataaatatgtacatatgtaaaataaaaatagtaaggatagttagactaattagatgctaaagataccaacttttaaatttatttcagtgtcattgtggaaaattttgaagcttttgggtttttgttaaacttataaatctcacttacacgcagcgtttttgaactcaaagtttagtgaagtatagatgcatcctcagttttctaatggttttcttctgacataggaagagaacctgaactattgttaactttgtttaccgattacatctgaattgcattcctctgttgttcaatgagcagtgttttgtgggatatgcttagataaataaattcatgtaaaaattacttatagttcaattaaatgtttgatttggtagccaaagagtatggaatcatagtcttgatcagtgtgaaattataggttagcgtcatcaacataaaaaccaagattctaagtcatccttgaacttcaaggtaattttcagagacccttgagattatgtgttagagatagggatgaaaaattgattttatcttttattccaacccaaatttagtagcagtaaatgcctgcagcaccatggtaagaaggactgcaaagctttcaggcttttcaggaaagaacactctagtactggctaccttggagtttaaggagacttacttttgaccattttgagggccttagcacagaactactcttggtcctagctggttagacaagcctagcttttctatgatcctccaaatgggatctgaataatccagttatcatgttagcattgaagataaagaactagtatattatatttattgggtctactaaaatttcatagacgggtagaattgactcttcagattccagaacaacccttcaggtcttggatatacaaactcctttagtgtagtgtccttgtgagcattgtctgtgggcgccaactttcaagtagttggcttgcagctcacaccagaatggaaaggacatgtttctaggaccctgaagagaattttcattgttcactgtttttatgcaaccaacaggatagtatgataattgtgtgtgttcatttaatccgtatttattgatcactcgtcttacacagtgtacttaggaatacagagataaatagaacacaggccctactcatgaaactcataatttgatagacatggcagtatcaataatttttgagtttgggcactacatagtcctcatgcaattgtttggctttcagcaagtcactttgagcaccagtttctttaaatgggtctaatggcaacattgctggttgagataatgtatgtgatatgtctcacttagtgtctgatacatggtagatgataactatcagtagcttacattttctagtacttttaaggtttacattgcagtttgacaagtaaaattgtattaaattcttatagtgtccctataagcttatattttttactttttcataaaccaagttaactggggtccagatatgttaagtttcttaagttcaagattgccaatcacgtcctaaaacttgtatttattcatacagctattccaacatgtaaatataaatttgttcaaaagaaatgagtgataagatatgaaatgagatggctttaaggaatgccgtagcacaacagaaaatcgtcaaatattgatgcctatgtggagggaagacaaagccaatgaactatgtttgtattaggcactgagtgatccaagcctttttattgttcttgacttagtccaatgagcagcaccagtgcctgcagtaatcagctgtttgtattatctaggagcccacttatagaattgggtgctgagatatcttattttgcattctatttagtagcctatgtatgtttggttagaaggagggaggagggagttgaaaggggagtttggatttcaagtttggcagtagtcattcacagtgagcaattttatatgccattattagaaatggaaatcagtcttgtagccatttagatcatgtgcaacaaaggcttttgaatatttttagttggttagttacttgctaaaattatgcaagaaatatgattttccctttatcttttttcacttttgggcttcttccattttgccttcaaggataacatataggtcatttctggaggaagaatattatatttgatagcttgatccaatgtggtaaactttaataaatactactgccccacttcttctatcaccctctcactcctgctattatccaggagaaatgtgatataatttctttcattagaattgaagggtgtttttatagtctttccattttttcatttattctcaaacattaggctgtgtaggtttgtaggttttctggccagttttgattattaagaatcacagcttttctaccatttaaggtcacatttatgagtgattcactaataaatctaagaactgcagtggcttgggagtaaatataagagaaatgtttctactgaaaagagaaacactgagaggcagaagtggaaggctatctggagggttgtggaattggcaatggtcagtgtttctgatccttaggtttgcaagcttataagcaattgaaaaagacagttattgaagacttaattttttctgaaagtactactgtttgattctatatgagcataattaatgatcatgctgaattaggaatttggtttgagggtttctataagaaacactgttggatactgcatttcaaaaatgatagaattttttcttaaatcttcacctcctactttctggatgctttttctttgataatatatctttatttgacccagttatcactagagttcagttgctaccagacttttcctaccagttgttgttggcatctgattccatctgtttactcatttattcatttcccgtaaatttttactccaaatatcccataggcagtgtgtcagaatatttttttttaaccagttgactttacatggcatttctttcagaacattctgccattcatttgtcaagtatttgttgaaagcttactgtgtgccaagcacagtaataggctatgaaacaaatgatcagtgaagttcaatccttatgtctaggaactcacaaattgggaaatttgggggatgaaggggagagaggttaagaaacataaagagacatataagcaaacaataacaatacatgttacctcttttttcaaagcacacttcataacttttctgttctctagtatctagcctttgtaatctttcttctgtactgttgtcagagatatttttcttagatgcagatctgatccaagttattctctgcatagtatacctatggaataagaaccaaacttcttagcatagcatgctggatatactgtttgctctccaaattctctctttaccatactctgttcttggggaggcagacctttatggattatattagctgagctcccttgccctttggtttcctgttgggtttagccaatgggatacggctggagattgcaaactggaaagaaagagaggtcagattatttattctcttggttctctacttgtagggtcattggttgacagtgactgcatcttcctgtatagctacagttgcagccactgtagctgccactgagtgccaataactcttgctctccagagacggattaaacgttaagataatgaaatttaaacttcagggcccctcacttgcaggggacttgcagaggccttaggaatctgtttacaaagctatttatttttgtaacatttgcaaaagttatttttacattctttctgaagaagggccgacggctgggcacagtggcttatgcttgtaatcccagcatttttggaggccgaggtgggtggatcacctgaggtcaggagttcgagaccagcctggctaacatggtgaaaccctgtctctaccccaaataccaaaattagctgggtgttgtggcatatgcctgcctgtaatcccagctattcaggaagctgaggcacgagaatcgcttgaacccaggaggcggaggttgcagtgagccaaaatcacgccagtgcactccagcctgggtgacagaatgagactccatctcaaaaaaaaactggggggggcgggtactaacaaaatggtataatcttcaggccctataaaactggaccctccaatgtccttaaccttgacccttcaagcttaggtaagtataaggtttacagggaagagagactactgaataacatacttgggaaggctattaatgaatatttcatggatgaaataataatttgagttggtgttgtaggatgaggagttcttcaggtgaagaaggatagaaaggtcattacaaatagaagacacagcctgttcaaagggaatgagtattttgatgtctacagtgaagcatactaggtagaaaacaaagaaaatacaaaagtcctgcggcaggaatatgtctgtcagttttgagaacagcatagagatcaatgtggctgtagacaaatgagtgatggggagaatagtaggtaaggttagagtttcctgttacttagggtcttgtaagccgttgtaaggactttgaccttttatcctgagtgagactgggaaacaggaaggttttgagctatgtggacatgatctgactattgttttaaaacaagtagtctggccactttgatgagaatagattggctgtgttgccacccaaatctcatctttaattgtagctcccataattcccatgtgctggggggggacctggtgggagataattgaatcatgggggtggcttcccccatactgttcttgtggtagcaaataagtctcatgagagctgatgattttataaggggagatctgatgatttctccttttgcttgattctgattttctcttgtctgctgccatgtaagatatacctttcaccttctgccatgattgtgaggcctccccagctacttggaactgtgagttcattaaacttcttttgtaagttgcccagtctcaggtatgtctttatcagcaacgtgaaaatggactaatacacagagagaccagttagaaggctattctagtaatttacacaagagatgataatgatttggacaagagagttgatggtagagttggtgagaaatggaaagtacagtattcaggatttgttgatggattcgatgtagggtattagagtgacagaagcgagtcaaggataactctagtatttttgtcctaagtaattgcaatggcaaattgctgtttactgagatggatgagactgggaagagcaagtttgaggaatggtgaaaatcaggagtttttttgtacgtgttaagtttaaggtgctatgttaatctgttctttcattgctgtaaagaaatatctgaggcagggtaatttataaagaaaagaggtttaattggctcatggttctgcaggctgtagaggaagcatgatgctagcatctgctcaacttctggggaggcctcaggaaacttacaatcgtggcagcaggtgaagggggagcccgcacctcacatggccagagcaggaggaaaagagagagtggggagatgctacacacttttaaacaaccagatcttaggggaactcactcactccctatcacaagaatagcaccaagaggatggtgctaaaccattcatgacaaactgtccccacaatccaattacctcccaccaggccccatttccaacactggggattacaatttgacatgagatttggtggggacacagatctaaaccatattattctgcccctggcccctcacacctcatgatcctttcacattgcgaaatacaatcatgccttcccaacagtccttcaaagtcttaacttattccaacattaactcaatagttcaaagtctcatctgagacaaggcaagccccttccacctatgagcctgtaaaataaaaaattagttagttactcccaagattcgatgggggtatagtcattgggtaaatactcctgttccaaaagggagaaattggccaaaagaaaggggctacaggccccatgcaagccccaaacccagcaggttactcattaagtcttaaaaccccaaaatttgactccatgtctcatgtccagggcacacgggggtgggctcccaaggccttgggcagctcagaccctgtggctttgcagggttcagcccccacaactgctctcatgggctgacattgagtgcctgcagcttttcctggtgtaccatgcaggttactggtggatctaccactttggggtctggaggactgtggccctcttctcacagctccagtaggcagtgccccagtgggggctctctgtgggagcttcaaccctgcatttcccttccacactattctagtagagttctccatgagggctccattagcagcaagcttctgcctggacatccaggcttttccatacatcctctgaaatctaggcagaggctcttaagcctcaactcttgcactgtgtgcacctgcttacagcttgcaccctctgaagcagcctcagctatacctgtgcccctttgagccatggctggaactagagcagctggaatgcagggagcagtgtcttgaggctactcagggtggcaggcactgggcgtagcccaccaaactattcttccctcctacgtctccaggcctgtgatgggaggggctacctccaaggtctttgaaatgccttcaaagccttttccccattttcttggtgaatgcaaatttctgcagcctgcttgaattcctcccctgaaaatagacttttcttttctatcacatggccaggctgcaaattttccaaacatgtatgccctgcttccctattaaatatgttccaattttatgtcatttctttgctcacacatatgagcataggttgttagaagcagccaggccagatcttgaactctttgctgcttagaaatttcttctgggttgggcatggtggctcatgcctataatctcagcactttggtaggccgagttgggtggatcacaaggtcaggagttcgagatcagcctggccaatatggtgaaaccctgtctctactaaaaatacaaaaattagctgggtgtggtgatgggtgcctgtaatcctagctactcagaaggctgaggcaggaaaattgcttgaaactggatagcagaggttgcagtgagccacgatcataccactgcaatccagcttgggcaacaagagtgaactctgtctcaaaaaaaagaaaaaaagaaatttcttcttccaggtaccctaaactatcactctcgagttcagagtttcacagatctctagggccagggcacaatgcagccaggttgtttgctaaggcataacaaaagtgactttttgcttcacctcccaatacattcctgatttccatctgagacttccttagcctgggcttcattgtccatatcactataagcatcttgatcacaaccattcaacaagtctctaggaagtttcaaattttccctcatcttcctgtcttcttctgagccctccaaactttccctctgcctattacccagttccaaagttacttccacattttcagacaccttacagcaacactgctttcctggtaccaattttctgtagttagtctgttctcgaattgctataaagaaacacctaagactgggtaatttataaaggaaagtttaattgtctcattgttctagaggctgtacaggaagcatgatactggcatctgcttggcttctgtggaggcctcaggaaacttagaatcatggcagaaggtgaaggcggaaccagcacttcatatggctggagcaggaagaagagagagagggaggaggtgctacagtcttttaaacagttagatctcaggataactcactcactcattatcacaagaacagcaccaaagggatggtgctaaatctgtcacgagaaactgtttacatgatacagtcacctcccaccaggtactgcctccaacactggggattacaattcagtatgagatttggtggggcacagatccaaagcacatcaggtgcctatttgacattcaaatgaagaaggtgaatagacaattggctatataagtctgggtagagtgggttgggagtacaaatggagtgttgtaagcatatagatggtgtctaaagccatatgactagatgagatactaaggaagtgaatatagatttttaaagggggagaaagaaagtgccaacatctgaggtttgggaccctccaacacatcagggaagtaggaagaactgacaagttaaagaagcagccagagagaaacagagaaaaaacagaaatatggtgatacagagagctaagtgaatgaagtgtttcagtgaggcagaggttgtcaacaattcttggtatatcaaataagataagtattgataattgaccgttggatttagcaatgttcaggtcattggtgatcttgatgatgctcagcagagtgaatttaaaatgaagtgagttcatgggaggagaggaattggaggcaatgagaagagacaacccattaggagttttgctgtaatgggggacagaaagttgttctttgggaaaagaggagttgagaagtttttgtgttttgttttaattattagtgttttaagatggaataaataatagtcatgtttgtatactgatgggaatgatccatcagagaaagaaaaattgctggagcaatgtctttgtccagtcaaggggggatgggatttagtgcataagtggagaggctggccttagataggaacatagacaattcatctgttatgacagaagggaaggtgtattatatggatataattcttgtacagtaggtgggaagatgtggtgggggtttttgaaaattattttcaaatttcttttttctcagtgaaatagaaagcaatgccataagttgaaagataggatagggaggtgttagaaaaaagggggaaaagtcatctaggagaatgagacagttaatacacaaggggaatgtagtatgatttctgggcagaattaaagccccacttgggattagtagtcatgaatttaaattgacatcagccagatatggtgtctcacacctggaatcccagcactttgggaggcggaagcaagtggatcacttgagatcagcctaggcaatatggtgacaacctgtctttatgaaaaatacaaaaattagccaggtgtggtagtgcatgcctctatagtttcagctgctaggaagactgaggtaggagtatcacttgagtctgggaggttgaggctgcagtgagccgtgatcacgccactgcactccagcctgggcaacagagacccctgtctcattaataatagtaataataataaagtgatatcagtcagcagccacattagctgcacagttgcaggtgcagaataagtagaaagttggcctttgctgagcaaataaaatgaagtcagatggaggaaagttgtcagtgtatacaagagaatgattgtgaaacatgaatatttccgattgcatttttcataatagccaaaagctggaaataacctaaatgttcatcaactaatgaatgaatatacaatggaatattagccataaaaggaaatgaagtactgatacatgccacagcatgaatgaactttgaaaacatcatgcttagtgaaaaaccagatgtaaaaggccacatatatgattccatttttatgtagtgtccataatgggcaaatccacagagaagataattagtgttatgattggggctgagtggaggaggaaaggggagtggctgttaataggaacatagtttctttttggagtgattaaaatattctggaattagatagtggtaatagttgcacaactctaaacatactaaaaatcactttagaaaggcagattttatggtatgtgaattatatctcaataaagctatataaaaataacatgctagctcactagaaatttgcttatcccaaactcaacaaattgaacagctcagaaatatagctgagctgtatttgtaatcaactaatgtaggactaaggtgaacaagtagctgtattacaatgtttgcagtctcttttcaggtttcaagattacagttgtttttttctcagacatcccttagtattaaaatgttattggctaagttgcagagcttgtgaggagagaccaattctggctcagtcttaattacttagtatcttcatctctccatcccttcctctccccttccaattaacaaacctttactaagctataaaaatcatcaagcactatcctaggtgctactggttatacaaagatggattggactttgtccctccccttgaatgtgaggtttaatggggaaatgaggtttaggaacttggagcacatttcatttttagggtgagactactctaatcgttcttcagcatcctcccatctatagcttatagataacgtatgcactcaaggcataagaaacttatttggatcttcattacgcttgaaacattcttccttttgtctctagaacatcagacattctttctcctcttactctaaagtattttggggctaccagatgaaaactcataataattttcttctgatgctctagacctgaaatatcttttataaaaacttcaacattcaaaattacgatgtatgttaggcaaagcgtgcatactggtgctatctgcaaaacaaataataatgtttaccttgcaggattgttgtgagggatcaatgagtatacataattgatatatggaagtgtcaaacacacgagctcttcaataaacattagtatactttatcactttgccaaagtctacaaacactaattttatatatggcaatatgttgagattgcagatatagacatagaccttaacagacaaaccctaattccaaagagtttgccattcattgatggaaattaattggttcagagatgttgaccatgtctaccttattatttaataacttaattaacttactacaaatctatcgatgttttccatcttggatttttatatcataaaaatgtagaattcttagctcatgactatatgaaaaatagatatttgataatgctttttaatgattataagctaattatattttgaatctcatgcctaactgaaatgtaatgttgcatgctggactttgaatttactaaaaagttcttttgttgtcttcctagaatggagctggtttgtcaaaatccaaaggaagccgaattggatttgatagcacacagtgggtatgtagaataaacaagaaatttctcaattataatgttcatttagttcattcatttactccgtaagtatttgttgaatgatggcaataataatagctaccttgtgtggtgggtggccggttggtagtggcaggtaagggacaggccctttaccaagtgctttatgcaatgtcttatttagtccctatagaaagtttaagaagtgagtaaatattgttactctcaattcacttagagagattaaacttagttggctgataatttggtaagaccagattctgtctgcctctaaaacccacattcactgagctatggtgtttccctaaatgaatgaatatatgaatcagatttatttgaataagggaaaagtaatgatcaggaataaaaatctattcaacctattcctttataagatgaggggaaaccagcaatatatacaatatatccttgttttgttttagaaatttcagaacctacacattgataaaatatattttcctatgttttaaaactaaatttagaaagaaaaacattgctgggttactaataaaacacaacatttattctgttagcatacattatgggaatgaccagatatttcttgatacacttcaatctttggcttctctataactagagatgtggaacactttaaattagaagtggattttcagatcaccaagcagtggtcattttagatcattgctaacaccaagtagattttgaactactgtttaaaagtaaagtctgggatatcctattatcaggctccccagctctctagtctataagtgtcaatgtaaacttttaatttattaaaaatagcaattgttttgctctgtgaatttagggtattctgaggataaaggtaagcatgatatacttggaagttatactacccagtcacagttataaagattttagattaaattaaaaagaggtattttgtatgcttctctgtaacacttctctacctccatcccacccttaggaaacacatacacctaatacttggacctgatttatcatcttgtggttgaagtaatttgctgagatttaaaattcagtattttaacagccaaaggcaacaggggtgatctttcatacattttaacattataagatgtgatgatacttagagaaacatatatttttcagatttgccatttattaggagtcttcatctgtacactgtaaagcaatttcagcaaaaaatttaaagccgtagtagcttcagttggataaaaggttttcctttatcggtattaaccaacaacattctgacaacattcccaaaccttttagtaaatagagagagcagtcagagaaagtacaggttcactgatacattttaaaatggaatttgtgaaaaatttaaagcttaaaataatagaaaaaagtagcgtgactctatccttttcattcaagaaatgatccttgaggtgggagaaaataatggatttttttcaaagtctttacttccacggtacgcaagcaaaaagttgaagagcagcttaccacattcagtgagttctctttatactcttttacattgaggggactaaaaaaaattgtaaatgtggtcactgaatgactatatttgcaaaatcacaggaaaggagaagtactaacatacttctaaacttttagaaggaataaaaggtgaaatctcatcaatagtgtgatattgagccctggtaaaattctagggctcaatgtttatggagttattaaacagatgacttgggagcacttagaaaagaaaatgatcataattaggaactaggcttttactaagaacaagtcctgccaagactttttaggttttaataaaattttaatacacaggcagatgaatgggctattatggtctcagcataatctcttttcaacaagatgtttttcagtcttataaacaaaatgagttactgaaggtcagatgataatagtgatttagaattaattggatttagaatcaactggacacgtttccaaggagcgttaatgattgtattgataacaacttggaggatgtgtttagaaggtgagttatagaatctctgcttgaccctgacctaatctgtatttatattaataatggtaatgaagctataagtgtgttcatcatatttgtatttaacaccaacctgagatccattcaacaaacattaaagtaccttttatgtagtagttctgttatctcatctttcttccaaaaccatttctttcttgtttttttcctagtataaagcacagaaagtaataaccctaaaagacacacacacacacacacacaaaatagctaaattggactattaaaattttaaacttctagtcatcaaaaaacactattaagaaaatgaataagcatgccacagagtagcaaatatttgtaaaacatgtatctcacaaaggaatggtatcaaagatatatgaagaactcccacacgactcagtaatagattttttgttcatgcctttcatcaagttgaggatgtattttattcctggtttgctgaaagttttaaatcatgaatagatactgaattttgtcaaatgcttttttctatattgaaattatcatagtttttcacttttttctgttgatttgtcaaattttattgattgattttcaaatgctaaagtaagctttcattcctaggataaatactacttggtcatgatatttactttccttttttatctttttttagttactggaattgattttctaatattttattaagtatttttgcatctgtgttcatgagggatggtggactatacttttttttgtaaggtctttgtcaggttttgctttttttttttttttttttgagatgaagtctctctgtcgcccaggctggagtgcagccatgtgatctcggctcactgcaacctccaccttgtgatctcggctcactgcaacctccacctcccgggttcaagtgattctcctgcctcagcctcctgagttgctgggactacaggcacacaccaccacgcccggctaatttttgtatttttagtagagacagggtttcaccatgttggccaggctggtcctgaactcctgacctcaggtgatccacctgccttgacctcccacagtgctgggattacaggcgtgagaagttttgctgttgagtatggcactggcctcttaaaatcagataggaagtattttctcctgctccattttctcagaaagtttttgtagaattggtattcttccttaaaaatgatagaattcaccagtgaactgtctaagtctgaagtttttccttgttgttttgagggcagtttttttttttcctaacaaattcagtttctttaataggtatagggcaattcagattttgtttcatcttgtggcagttttgttaaattgtatttttaaagaaatttgtgtcatctaagttgaattttttggtgtaacattgtttatcctaactttttacttagctgtttctcacactgaggtaataaacccctataaggcagagattattgtattcttggcatttgcataatactctacactaaaaacaaataatgagactgattcttagctttatctcatcctttatccttacaattgatattttgtctatttatttatcttgtatatatttttatgagttccttcagattttctgaataagaatttattcttaatttcatgaagcacctttttgataggcaaacattcctataagtcttgctttcattgaagtaggcttttaagcaatagtgtatgccagatattctgtttatccttgctgttcttagatattacttattcctaagtgtgatttagtccattttcattctactgttgaatttttgtttttttcagtaggggaccctacttactacccagcagagttatattttgaaatattgcggtattagaaaagcacattatatatggcagtcatcaagcaggcagtgtattttggtctgagtcttttgcttagaaagattattaagcagcattacagatatgaagaaaaatggtacaaacaactgaattttgtttttgaaagattaacaagactgatttttaaaagctgacggatagttctctcaattttgcttgaaaagatttagctaatactaagagaataattttttaagcaccacattttcatgtcagataccacttcctctgtgaaatttcttatccttttgatgtatggtaaatttgtagcttactggtctgtacttttataatatgttgtatatgtttttcttgtagcatatttcaccttatattgaaaatgttcatctttcttagaagactgcttattgagagcagagaccatatgtgctatttaatcatttgtattttttagcacaatgataagcatggtatctattgggtaactactctgcattcttatacaattaatgaattaaaatgttataaaatagactgttgtgttggcttactggaattacgagaattctttttctctcaaacagcgtgcagttaaaaaatttattatgttaacatccaaccaaaatgtaccagtgtttcttattgatcctttgatactggaattgattaataagaactttgaacaagtcaaaaatacttctcatggctctacttcacaatgcaagtttttctgtgttccaagagactttactgcatttgcactgcagtatcacctatggaagaatgaggtaagtgacttgctttcagataatggaatgtgtctctttttacaaaatagtataggtttaggctagtttaaaatgtaaaacattaaaaatttttcctgaaacactttataaattgtatcaggaatattttcagctataaataacaatacaactaatcactaaggcaaataggggatttctttttcttatataatgagaggttaaaaggttagtggctattgatattagtttagctagccactgatgtcaggacttgtgtctctgaaattctttattcatttacctcattatcacaggatagctgtcgtagctccacatatcacatccatgttcacaacaggaagatgagaggaaagattctgcttttttgctgggggaaacttctcaatatcggtatttttaggtcatttctgttgaactgtttgatatctcatagaaaaagcctacaaggcttatttttacaaagaatattttataatgtccctttatattccccaaatgaagttcatagaaattataaccctcctatatacataattccccaaatcaatataatgtattaactataatataacctagaaataaaaggaaatgatatgtattgctgtgtgcagatgctccagaatgactacactggaagacataataaagtaattcagatgcttgtatttagaagtaggatcacagaatgtggtagctacaaatataaacccatactatgaatgatattgttgttggcaatatgattttccaaaatagtgagcaagtttccaacaacaaaaaaagtaaaattgtctcttcattgacatgactattgtattcctgagaaataaaagctcagacaattataaacaagtttttcactatgtgattatgtgacaggacatttgaaattacatagtacacaggatagattttcatattttggattgtaggatatctaatgttcttggcctaggactctaaatgccagtttgtcattatgataaaccaaaaatatccccccaaatttctgaagtatctgttgggtacagtcccacttgccttgagaaccactattttagaagaaggggagtatgccaccattggcaaaactgatactaccatagtcaagaggaagaagcaaaagctcagccatacccagaatcagcacatgggttcaagtttattcttcgtttgtttttgtttgtttgtgttgggttttttgtttttgtttttgttttttgagacggagtctcgctgtgtcacccaggctggagtgcagtggtgcaatctctgttcactgcaatctccgcctcccaggctcaagggattctcctgcctcagcctcctgagtagctgggattacaggcgtgtgccaccacgtgtgactgatttttgtatttttttttagtagggacggggtttcaccatattggccaggctggtcttgaactcctgacctcaaatgatccacctgcctcagcctcccaaaagtttctccttttgtacatatgacatcctactattcaagagattcaagagcccttggatagtcccccctaaaacatcccccaatgtggagctaatcagattgttagatctaataatgaaagactccatttgcatgtgatttttctttattaatgccattaccataaagtgagcaaacctctgccaaggctactgggagtggacttttctagcaaaaccttgacctaggcctttacaccaattgatcagagcaactattttgttctttacttctcttgttgatggttataagaaagcaaaccatatcataattctgcctattttgtctgtcagtctttcctcctataacccaaggtcacgttcttctcaagttctggccggccttttaaatatttcctgaatttgtcagctgataatgcctttcttttattctattcagtagtgtctttctctgaattggctaccctccccctcagtcagtgctttctacttctaaggtgtaccaagaaagaaaagggaagaagggaatgttacagttgataatgaaacaaatgatgttggaaaatgaaccttgtcttacagtatgtttgttaatttctaatgatttgcattatgatggtgttctattatggtagtattttaagatgttgggatgtaaactatgagatgaaagaactacttttttgaagtacttttgaagataaaggttattaaaagttaaattaagaattacaagtttaattttaagtgctgtccttaaatcaacatttactttatagaaactaactggaaaacactaacatgagcattctcattccaaggaagggatttgtattaattttcatagagttttttttgttttttttttttgagacagggtctcactttgtcacccaggcttgagtgcagtggcacaatcttggctcactgcagccttgatctctcaggttcaagtgatcctcctggctcagacccccaagtagctgggactacaggtacatgccaccacaccttggcaaatttttgtttgtattttttgtagagacaggttgcccaggctggtctcaaactcctgagctcaagtgatccacctgcctcagcctcccaaagcgctgggattacaggggtgagctatggtgcccaacctataaagagagtctttggctatatctttcctgctacatactttgtatttttgctgctttcctttattctcccaccactaccttctgcccatcaccctcattaaaaaatgttcttacagagcagattagcacaaaaatatggctcaagttcaatataagaatcactttagttttgctactagtatttggctttaaatattcaatgtttaagtgttgtttcttgatgtttgatgcttctttggttctaggaaggctggtttcggatagctgagaatatgggatttcagtgcctaaagattgagagtaaagatccccggctagacgggatagactcactctctggaactgaaatccccctgcactatatctgcaaactggccactcatgcgatccacttggtagtctttcatgagaggagtggcaactacctctggcacggccacttgagacttaaagaacacattgacaggaaatttgttcccttccgaaagttacagtttggtcgttatccaggagcttttgacaggtaagttcagagtcaaaacgtgaaatgtgaaatgagtgttgttcagtcataattcttgcagtgtttttacatttgagtattgaaatctaatatataatttatataagtatttacagtaacattattcttaatgactccaaattagaagccacccaaatgtccttcaacaataaaaggattggctgggcactgtggctcatgcatgtaatcccagcactttgggaggccgaggtgggcagatcacctgaggtcaggagttcgagaccagcctggccaacatggtgaaacctcgtctctacaaaaaaatacaaaaattatccatgcattgtggtgggtgcctgtaatcccagctactggggaggctgaggaaggagaattgcttgagccctggaggtggaggttgtagtgagccgagattgtgataccacactctaggctgggcaacagagcaggactttgtctcaaaaaaaaaaaaaaaactgtaaaggaataaataatttttgatatatgtgttcatacaatgaagtattacacagcagggaaaaataaactaggggtctgtgcacattgtggatgaatcctacaatgctgaatgacacaaggcacaaaagaatctaaattctattattattattatttttttccattcaaaagtttcttttattcattaataaacaatgatatatatgtatacacagcttcataatcataccaaaaaagtttaagtgaactatcctttaaaggctgagaccataactttttgaacagaaataatatggattataagacagtatattgatttttgctgtctttattttaatataaagaacaaattgtgtggtaagactaatttattttcccactttgaaattaaacctctctagaaacatttagataaattatgaactaatctttaaaataccgtattacttcagcatttcaaaatcagtaagtttggaaactgtatttaagttaatattaggaataatataaccactgttgataactaacaatatagccaaaagaaaatgtggtacatacacacaatggagtactattcagccataaaaaagaatgagatcctgtcatttgcaacaacatggatagaactggagatcattatattaagtgaaataagccaggcacagaaagacaaactttccatgttctcacttatttgtgggagtgaaaaatgaaaataactgaactcatggagatagagagtagaatgatggttatcagaggctaggaagcatagtgggagaaagaggggaagagggggatggttaatgggtacaaaaaaatagttagaaataatgaataagactgagtatttgctaggacaacaaggtgactatagtaaaaaataattgtacattttaaaataactaaaagtatacttggattgtttaatacaaaggataaatgcttgaggtgatagataccccatttactctgatgtgattattatgcattgcatgcttgtatcaaaatattgcatgtaacccataagtatacacacctactatgtacctacaaaaattgaaaatacaaaagtgaaagtaaattctattattacttttataaaaagttcaaacacatgctaaattatgttcatggatgtatacccttatagtaaaagtattaagaaggctaagcaagacgtaccaaaaaagactagatagaggacacagagaactacagggaaactggaagaattttatttctgtggtggagactttggtgtttactttataattcattattttgtgcctttatgttatgcactttcctatatattttttaaaaccatgtgcaaaaatttatctttggctatctcaataataaaaatatttcttgtgagaaacagttatttgaaggaactcatgtaaaatttgattagctatagtttataatattaacaattacaggattaaaaacattcttgaagttatacttggagtatgaagtttctaacctagaattgttccttttattctccttttgaaatcagcgataatgatgttacagtctactttgaatagcagaatctgatgtaaaggtagcagtaaatatttgtaaggattttcacattaaaaactccttcttagtaacttccagtgagataattcttatctgttacacttgagaagtgtaagagtatgtttattcttgccttcttttaaaaatatatatatatattatatatatatgttttctctctctctatctggaatcatgtgagattgccttcttattagtacttaaagtcacatatttgagaatgactgaaaaaggtattcgaaactgaagtcttctatattttttgtgtatgaaaagtcggaacttttctgaaccaagccatattttcaaaatgaccaaaaaaaatgagtagagatggagaacaatactttgtttttattattggcttctcttattttaatcaaaaatcttaatactcactgttctcttaccacttttttgcctgtttttttcttattctgtatttcaaatgaccttctttagggagacattatcttttagttttttaaagctttgtgaatttatttcaaaatttaataacttagtaaagttcaaaattgtcagttacttattaaacataaacatgtgacaatagataaaagctatctctacattgtaaaattttatatgagtaggaatggaaaactctcaaataatatttttagagtatgggatccaaaatacataagatagatttgcagattagcattttacccattaatgagattctcaggccattgtaattaacttgtgtgtcttaagtgttaaaaacatttacttctctaaaagtaaactgataattaaaaattatgtcacaaaatttttgtttctgcttaaaatgccaagtgtgtatgaacaagtacaaatatattaatatataaatacattaaccaaaataattaaaactcaactgtttgatgtcagatttttcaaggtcttattaaaattgctaattgatatctgacataattgatgaaactatgcttgatgtttaggtattttgctaatgtttgatatttgtaagaggctgccagtattctgggttaaatccttttaataaatcttttattattattattattatttttaaattttactttaagtagtgggacacatgtactgaacgtgcaggtttgttacataggtatacatgtgccatggtagtttgctgcacctatcaacctgttatctaggttttaagctctgcacgcattaggtatttgtcctaatgttctccctccctgtttcccccacccctcattaataaatcttaacttttgttttcaggccagagttacagcaagttactgttgatggactggaagttctcattccaaaggatccaatgcactttgtagaagaagtaccacactctaggtttattgagtgtaggtataaagaagctcgagcattctttcaggttagagacaaccaaatgtgtacttttaaattaaagaaaatgttgggattatttttaatatttgagggtggtaagatgaaggggcttatggaaaatagaaaagtaaacatccttttttgatatgtctcttttcttctagattgttttctttcagttttttttagaagtagattaaaaattaaccttaagaaactattttctaagtcaataggttgatatttatttattgttttatttgaataactttaatagatttagcactggcttctgccttaagatagcccattaactttgtgaaaggtggtgtattctcagtccaagtaggataaagccactatagaagatggaccatgtagatttagaaaagacttcatgaaaatacagtttgtttcagagttggcattgaatataattttttttgcatttatgaaggtttttgaagataaatgctacacaaagaccaggtgcttttaaaactttattctcttgctgcagctttcaattcaatacacatttattgtgttccgcaggcttctggccctggggatataaagatgattttgaaaggcatgaaagttcagctctaagagatgacatgaaacacagagatacagtgaaaacaggcaaatttacagtggggttttggtacctgaattctttcacttgccctttattttctggggttccctgccaagaaagctgtgtccacgagggatacgaaaatgaagtatataactgtcaagtgcccaagacccacaaatctgaggtttctctaatacagtgtactggcacctaaagctgaggcctgacagcccaagtgggccttcgtagccctatttccttaagtcattgtggagctgtgaaatttatgcagccagcctcatgaataaaaagctgaaaaaccacatgtgtggatgggcctactctagtagaaaagtgctgcctgacatatgcctaccacataataacaggaagtagaagagatggagttttgtgcttaaacttgaccgctcttcctgtcctaagggagtttgctgtggttgtcatctctattatagcaattatcacagtgaattatgaatatctgtcttgtcctcttatcaagttttatgaacttcttgataacaggagtgttcttttatttacctgtgttggcccagtatctactgtacctggcataaagaaaagatccagtagggtcagttttcaaattaaagtgaacatacatgtatttgaacacttgatggcgccaaacagtcttaaatgtaatgcttggtgtaaagcaataaattaatctaatagacctcatcaagcagccgcctttctttttttaaaataatttttaaaaagcaattttaaatacataaaagctgcaagtacagtaccgataacttttttttttctgaaccacttgggagtaagatgttgaccacaacttcaaaaaatttagtatttttttaaaaataggaacattctctacatgtcctaatatgaaagttaggaaattagcacatacatttttaccatttaatccctattcaatttttgtcagttgtctcaataataacctttgtaataaaaagattcgattcagaatcacatgttgtcttaattttcctgtctctttagtcttcttcagtctgggacagtttctcagttcttttattactttcatgactaatactttggaagattacaagccagatgttttgtgcagtgtccctcatttggggtttgtccgggggttcctcatgttagatttaggttatacttctttagaaggtatagaagtggtgctgtgttctcattacatctcactgggcactgcataattttgatttatcccattactgttgatattcacattgttcacctgattaaagtgctgtctgaaacttcgtatctttaccactatgaagtttctgtttttccctttataataataagcatctggcaagaagttactttaaaactatgtaaatattgttttcctcattacattttcaatttatttgttcatatcaatataaataaattcatggtttcctattttaccctatgggttatagtcaattattttcattatttattttgatcttcagattgttccatatttggccagtagaaactccttcataatgctttctgtgtccttttgacttgtctccgttgttttttgaacactttagtactttttggcactataaaatattctgggttcatcttacaattttcatacctccaccctgggatcagccatttctttaagtcctgtttccttttagaagccaagacctggatgccaggtgtacccattgctatttgggttttgctgcagagagtttctctcagtgaacaggggtagggtgtatatgtctgtgtgtatttatttctgtatctatctattgaaacctctgaattcacattgacatctccagtccggttaaaagttccaattaaacaacagagttcatttccatatttgcgactcccttttcaaatcgtgagaaatctgactcccattgaccttaatgtttacttagttgttcagtctccctgtatgtaacctatcttccaacacatgtcctcccctccctaccccctgttcttctcaccctacctgggcactgctatcctctgctgggctgcacacacgtagaggcattcttcttaccctgttcaggctctgacttcccacacctggctgctgttctgcagagaggctttcctcaccctgcttgggctctgactccccacactggacactctcctactctcttcatgtggatgtcctcattacctgcctaggctctgataccccatatcaggcaatccctttgcacaaaaacctttcttgctctgccccatctaatggttttagtatcgaatagttcaggaagggcgggagactttatttacttttaattattttctcaatctaccatgaagttcaaaaactagaataatataccttttcctgaatttgattttgttttagcaaaaaccatcacaagataattaatgagctccaggctgttgaatatcagtgaaaaaccaaaaggaaagttggaaatacctgtacacctggcctaggaatatctagataacaatatttttattttatttctactaatttgctctaagattttgggcaaatttctgagccttggtttcctcatctacaataagagttggtaccttctgtcatcttattctttgatataaggtttgtgcttttggattccacgattcttcttgggctttgtgtccccgttcattggctgaacaggaaaaattaaataaacatgatatttaaagtaggatattaattttgtctttttttagaggtatagtaatcctgagatttgtacttgggatttatttttatttgtttacttatttattttatttttaacttgtaagttcaggggtacaagtgcaagtttgttacataggtaaacttgtgttgtgggggtttgttgtacagattatttcaccacccaagtattaagcctagtacctattagttatttttcctggtcctctttctcctcccaccctccaaaagaacccattgtgtgttgttcccctctatgcgtccatgtgttctcatcatttagctcccacttataaaaacatgaagtattaggttttctgttcctgtgttagtttgctaaagataatggccttcagctccatccatgtccctgcaaagaacatgatcttgttcttttttatggctgcatagtattccatggtgtatatatactacattttatttatccagtctatcattgatgagcatttagattgattccatgcctttgctattgtgaatagtgctgcagggaacacacacatgtatgtgtctttataagagaatgaatgatttatattcctttcagtatatacctgataatggaattgctgggtcaaacagtatttctgtctttaggtcattgaggaatcaccacactgtcttccacaatggttgaactaatttacactcccaccaaccgtgtataagtgttcctttttctccacaacctcaccaatatctggggtttattttattttattttattttattttattagtttttttttacttgttatagtagccactctgactggtattagatagtatcgtattgttttttattgcattttctaatgatcagtgatgttgaacttttttcatatgattgttggccacatgtatgtcttttgaaaagtgtctgttcgtgtccttcacccactttttaatggggttgtttggttttttccttgaaaatttgtttaagttcctgatagatgctggatattagacctaatagttaaggtttgcaaaccatagtttgcaaaaatgctctcccattccataggttatatgtttactctgttgatagtttcttttgctgtgcagaagctctttattttaattagatcctatttgtcagtttttgcttttgttgcaatttcttttggcatcttcatgaaatttttgcctgtgcctgtgtcctaaatggtattgcctgggttatcttccagggtttttatagttttgggttttacatttaagtctttaatctatcttgtacaggatatttttaaatgaaaaaagtatgtatactataatttttaaaatttatagcagatgtttaaggtatatagctctatgcatgtatgcactttaacacatacaaggatcagttctgagaaatggaatttctggctgggcgccatggctcacgcctgtaatcctagcactttgggaggccaaggcgggtggattgcctgagctcaggagtttgagaccagcctgggcaacatggcgaaaccccggctctacaaaacacacaaaaattagctggacatggtggtgtgcacttgtaatcccagctacttggaaggctgaggtagaagaatcacttgaacccaggaggtggaggttgcagtgagccaagatcatgcccctaaattccagcctgggcaacagagagaggagactttgtctccaaaaaaaaaaagaaatggaatttctgagagtgtcatgttaagaaaagtagattggggtgggaatatgtccatatgggagcagtaccagcagcaggtaactatcagacctgatgtttttgtagagcacaaatttttcatatttgctgtttagtcctttcagtcactctgtgtaataaggcaaggattcttttaacaggtaagaaaattgatgtttcaagatgtcagttacatggtcatcattggttgagcatggactaaatcctaggtctccacctcttaactccaggcttttcctactacaacaagcattataacatgtatctctcattccagtcatttattgtaagagcacttatggctttgaggaaagggatgtattcaaattgaagggatcctgtgtaatttgtatattctgtagacagtgacttatctgcaagaaattcttcttactgaaggtagggtactttttgcttaagattcatatagtccatccaggatctatattctttcctactatattgtaaaagaattacaggatattttaggatgttgcaggcctgggaggggcttagtcaatcatttattcatttgcccattcatcagtatgtgtttttcagatattatgtgccaggcaccattctaaacctgtagatacagtgatgaagagatgtagtacttgccctcagggaactatctttacagtctagtggagggaatataaaattgatgattaggaataaatatgatatgaattatagtaaaagtatttacaagtggtaactattataagcttgttaaggaaaaagataattcatttgtctttgtatatctagaaccaaacataattctttgctctataaatgttgaatagaaacacttcctgaataggaacattggaagaataaatacatatgtcttcctgggaaaactggggaatgttttgcagaggttggagctgagacttgaaagattttattgatcagggccatatcagacaaaggaaacaagtgcggaggcttgaaaagttgtggtgtatttgaggagttacaagttattgtggtatatttgggggtttacaagttataagatgaagtgtgaggagatgcagatgaggctggaccccagtagtcaggaaccagaacacagtgtttatgtccaccaggacaagaagtttagattttgtcccacaggtagcgaagcaacactatagaatttatagtgctttcctcagctccagaacactctaaaaacgaagagaatcagaaaaccaagatgactaaatgatatatatgacctgacaatttgcaagacatttttctccttcaatcttcacagcagtcctgtgaagtataataattatctttaaactacaaatgagaaaagtagatacaagagagatttgtttattacattctttcattcattcagcaaatactcaggcactactctacccactggagatataatgataaaatgaatgcactttcctcatagaaagtgaggatgatatgtacatggtcaaagctaaaaagaagtgcactagatttgataatctgattcaaaatctcaggctttttctactatactacacagtctctaaagaccaatagaatcactgaatggtgaaaacattattaaattctttttgtttcagctatgtttgtagctctcataattagctttattttatcctgattgtccagctactaaattgtgatgtaaaggagggagctgataaaaggatgtctcatcctttgggaatcctggttctattctttcccttttaatttatctctccaagaatctgctcttaagtgttcattttaatgtgggacaaacaagtaactgtaaaatgtggtttttataatataaaaagattatatggggttagttttcttttttttctcctttctttctttttttttttttcttttttgagacagtctcattctgtcgcccaggctggagtatagtggtgtgatctttgcttactgcaacctccacctcccgggttcaagtgattctcttgcctcaacctctcgagtagctggaactataggcgcgggccaccactctcagctaatttttatgtttttagtagagatggggttttgccatgtgggccaggccagttttgaactcctgaccccaagtgatccacctgccttggcttcccaaagttctggggttacaggcgtgagccactgtgcccagcctggggttaattttcaaatttaattcagatgccacagaaaggttcctagcaatttagaaatggctgtaatagctgactatttattatatctgtagcagtaccttgatgataacactgtggaagctgtggcctttcggaagagtgcaaaggaattactgcaactagcagcgaaaacattaaacaaattgggagtaccattctggctgagcagtggaacttgtctaggtaaaattcttacgactttccatttgtctttctgtcattttgtcctctggctttagggattactgcttgagatgacaaaatatcagtgacatttgaagtgtcatgtgtatagacagaataaacatgagtgcatgcagcaaggatctattgatttccttaaagaaattaatttgagaattataaaaaagaatgttagaaaggccatggttgtgtttactcataattataaataatatgtataaaatgtatatcagaacatgtagactatacaatagtccccccttatccatggacaatacattccaagaccaccagtggatgcctgaaatctccgatagtactgaaccctatatacgctgctctttccctatacatacatatgatgtttaatttataaattaggcacagtaagagatgaacaacaataaataataaaatggaacaattttaacaatactataataaaagttgtgtgtgatctctgtctctcagagtatcttattttactgtactcactgttattcttcttacgatggtgtgagatgataaaatgcctacatgatgagatgaagggagatgaaggatgtaggcattgtgatgtagtgttagtctactattgaaaatttcctgggaaaatcaaggaatgtgtcacagaggctaaatctgagccctgaaagatttgatttaacacttctgaattgtttatttctggaatttaccatttaatatcttcagatcgtggttgtccacaggtaactgaaactgctaaaagcaaaaccacggatatggcaggactactatagttgattctcagataatccttaaattagcattttattatttctatcccaaagattgttattgcctttttttataattataaaaaaccctctatttctttacttatataccattcaaacagcttgcattgcaccaaatgtttctactgagaggaacattaaagacagtgtcataaggtcttccatcagcctttcctaggtcattggtagtatcactaactagacatcactgttcatctgacatggacatacagacttttctacagtccttaagcaggttgctattagaatctgtgagtgatttctgggtctctgtccactgtccattaaatcaaacttctttggaatttagaattatttagaatcttaaattttgttttgtgtttatttgttgtctcttgattatcatgatagttaattatagctgtatttgctttttctttatagtaaccatatctgtacaaaagttaattcaactcctgcctttatagggatagggttgccatccaatttattgttcaattcaagagacttgagagtgaaaggaagcaccattaataattatgttggtacaacaggcataaactgggatatacggttatcctatctattagcctttgttgaaaatttacatggttcttcctgccaaggagcttactactagaataagccaaaaaaaaaaaaaaagtacatctcacacatttatgtgatatttgctttaaggtttaattttttagaaacaagattgttttataatgtgtgtcatcaaagacacttcatagtcatttgacatgatttgttttgagttttcagtcccatggttttctgtctgatttaagggcacttatgagggagttgtattagatgatatttaagaaaacttttatttttaattgtttataattctttaatagaattattttagaattccaaacaatattatccaacagcaatgcctataaggataatcgcagtcatttatttacttttgaaataattggaatgaaatgattagaaagatcataggggagacccaggagtccttaataatattaaggtacatgttttatttcttcagaacagtgctatagcaatgaattagagcacatacgtggtaaacacttagaaatatcatttggcagtgtgttgaacattgaagctgctactgcttttctttttcatacggcccatcaggtggtcactgttgagagctgttaggttctacaaattattgctcaagaaaaatatattggttaagcaaaagaattaaatattttttgcatatcttaacagccccctctatcactagagattaatgattaaacattcttatcagcaacttagtgttattaaagctaatggtttattcagaaactaaaatatatcatgaaagtttttgaggaagctgagagtgctcagacagtaaaaatagatacatagatagatagaaggttcaggtgactgctcaaacaaagtcatttagtttgaggtttaatttttaaaaataattttggtgaagcatcttaagtctaatcctgtgaaataaaatccattctatagccccagccactcaagaggccaaggcaggaggatcacttgagccaggagtttgcgtacagcctgggcaatatagtgagactctgtctctttaaaaaaaaagaaaaaaaatccttgttacaaatataatttgttataataactaattttttccaaacctaaattttgttaaaaaaatttaatcttctttttaggatggtatcgacaatgcaacattattccttatagcaaagatgttgacctaggaatttttatacaagattacaaatctgatattattttagcatttcaggatgcaggacttccgctcaaacacaaatttgggaaggtcagtaacaaaagtcggcttcatttcataagtaacatatctcacttgtaaagtttacattaagcaactcagatatggttaagaatgctacatacataattttatcactcagtattgactaggatgagttcagcagaagcctgttaccacttgtaatttctgcactgtctaggcaaaagcaagaaaatctggctttctactgggttggtgcaaaagtaattgtggtttttgccattacttttgcaccaataatgataagaaaagaaggatcttgaactcttataggtgaatgtattgctattatattaggcaacaatgtaatataaaatcaatataatgtataatatacaattaataagtaagaatcccacccgccgtacctgattgtttctcatgagtcatttaatttacagatgtcattatcaacataaaatattccattgattgctaagggatagaaatatagaatcatttcaaataagtacttcaatttcttgtttatcttatatgtcctaggctatagcagtttgctcagacatcaactagggataggtcattggggcctagatgaaatctccctctagacaatttgattcctatgccctaagcccatgatctcttgcaatcatcttgttcttaatttgcttgtcccctcggaggtgttaccctacaagcaagtaaaaatatgtttagtcggctgggcgcggtggctcacgcctgtaatcccagcactatgggaggccgaggcgggtggatcatgaggtcaggagatcgagaccacagtgaaaccccatctctactaaaaatacaaaaaaaattagccgggcgcggtggcgggcgcctgtagtcccagctactggggaggctgaggcaggagaatggcgtgaacctgggaggcggagcttgcagtgagctgagatcgcgccactgcactccagcctgggcgacagagcaagactccgtcttaaaaaaaaaaaaaaaaagtttagtcaccagaaaattattttttccatcataaatagttattttatgttactaaaaaatataaataaaatattttactgaggtcaaagtcaaataacagagctctagttattcagcaaacatttaccaaacattcactataagtatggcactgtcctctgcacctgggagacaaagatgaataaatgatagttcttacccttgagaagctcactgtctaattgggagggggaaaggctgcataaataattctgtgatgagtgctgtggcggacagatgtaccaagtccaatgggaacgtaattatttgtatgataagttttctttagggaaatgttctcagaattatttatttttttaccttaacttttatttttttcttttttccatgtgtgtagtataatgagctagactatttatgtatgtggctatgaggaatgccactttacttaagtacttattgattgttatgagagacttatttcctgatagttttatttggattattaaaggaaataatatttctttggttcttttccttttttagtcagaaagctgctctggaataggatatttctattttttttctgcagtgataattaccataagtcatttactctgagttatcatcaattgtaagaaacattattttagatgcagttaagaaattaaatgatatgttactgatgcatcccaatttcagaggtgccttaacttgaaaaaatgtgcatcttagaatgaatactctatgtatgtaaaacttaagaatctgtttctttatttttattttttaaaaaaaggtttttaaaaatgtatttcctttgtttcagtgtgtgaaggttttcatcttccccataggtagaagacagcttggaactatccttccagggaaaagatgatgtaaaacttgatgtttttttcttctatgaagaaactgatcacatgtggaatggaggcactcaggccaaaacaggaaaaaaattcaagtatgaatcaaataagtacttatttataaaggtactacagaaataatttcaggaggtagaaataaagaagtaactgaaaagaaaaccaaaaatctctttcaagactccattattagctaacactttcttagcttacccatagagtccagttatgcctgtgaagtaagaatacctgtaaggacggtttgtgaggaggaagtgtccctgggtttgtcagtccaagttgatgatacagctggtctattctcagttctgagagagagaatgagaatgagaacctgaagagcatgggttttagagtcaggctgacctgggaaaccttagctccaccctaatttgtggcctttagattttctgaacgtaatcattttatccattacattgagtaatactactgtgtgtcaggcactattctgaacgttttacatatattaacccatctagtcctcaaaataaccttcagaggtagatattctgaagccagtgtgattgctgttgaatctcagctctttattttaccagctatattaccttgagcaagttatttaacctctctgcctaagtttcctcagctgtaaaatggaaattatagtagaaattgccacatagagtggttttaaggattaaaagaattaatacacaaaaagagctttgaggtgtgtcaggaggtcctgggtgctaagtaattattacctgctgttactaatactactatagtagtagtagtagtagtagtagtagtagtagtagtagtagtagtaaagaaaactatttctcttcttattctcatgagaaatttacagattagagacatgtataattatctcaatattaaactgttacatctattcttagagaacttctgtaagagtgtcaccttttttctaagaaagataatttctagagccagtattagagtcctgttattcttaaattactttctaaggcttgaattttttctctcactgacatgatccgaaacctgcaaacctcaaaagaactgttcatttccaactactacatttctggagagaaaaagcttctttcattctgctttaacagctctttatagtagcagtgtttgggaagtgtgaagtgttctgattatttaacaagagaaatgagcagtgatagaactgtctggacagatggtgtgagtcccagattttctatcatgttactgtgaccttaaaaggcagagaaaagaacaggagatggctgagtagagtagtttctttggaagattcccccagccatatgccatttttattcttttcggcactatttactttaagaaaatgtagtatttttaacactactattccttggggatgaagaaaaacaaaatgtttaaagctagttcaagggtctttttaatgtattttaaatttttgaatagattatacattacatagttaaaatattcaaagaatataaaggatgtgtatgaaaagtaaacctttctccatcctctgcccctcattttcccgtttctagttgccctttacagagataaccatgattactcatttcttatgtatcctttccgagacaaacatatgctcgtatacatatagtatttacgttcatctctccccctttacacaaatagtattatggcatattacacactgtctgtatgttcttttcctcacatagctatgtatcttggaaaatgttccaaatgagtatgtatagaaatagctgcattttattccattgtatggcaataccataatttattcaaccaattccctattgatgaatatttaggctgtttccagtagtttactgtgaccctcagttctgcagtcactatctctgtccatatgtctttatgcacacgtgtgaaaccctgtgcaggataaagtattagactcaaattttggggctaaagggaatataagcatatttcaattttgatagatattgccaaattgccctccaaagatgtttccccaatttatattctcaaccacatggtttgagaatatgggtttattttttaaaagtgcactatctgtaaagagaggtaaacttgctcaatatttgccactaatcagtaacttatcaattacttgtaatcagtaactaaatctaccatacaccaaatataattgggagcacattagaattactgttcaaactagtcagtataatgtatcatctcaccttctccaaaggtctttttgtctttataataacctattttttattttatatatagttcattctgagaaaagcttaataatatagaatgcttactattttttaaaaggcagaagaggaactcaagaaggaagaaaaaagattttctttctaaactactctgcaggactatagaatgatatctttggtcctaagatttaacagtatattaagagtaataaaaaagataaagcttccaggatatctgctacctatcaggcactgtgataggtagttcatatatatatttatatatataatctggttaatcctcatactatccctgtgggttcggtattctcacctccagttagacattaggaaactaaagctcagagtgaagtaacttactcgaggcttttgactgttaatggcaagatcaagatttaatgccagacctgtttgacccctaagcctaaatgctttcttcttagagttaataggttaagtgagttagtacatctaatgcatttagaacagtacctggcacattgtaagtattgtgtaagtagtagctactgtcagtactgtattattattattactgttactgttattataattaccatgctgcactggcataaggtatggtactttcagcacagtggtaaattggattagtaattttctaggcaggcatattttcttcctccatctcatgatactcattccgtctttagttctcaatctttcacttctttataggaagcccttcttttacctgaaatccaaattccatttaaaaatattgactggattctttattctgtttttctccagcatccaaatctgccagtaataaaagtgatgaatataataactatgcctccagaatgtgaagttcttaattcaacttcacatttcctaaagatgctgcctagatttatttggtttgcttctttccttcccattttgaatcaactggtatgggtagaagccagaagtttgaaaggtaataataatagttaactttattgaatacttactataagccaatcaatatgccaagcttttatatgtgttatcttatttaatcctcacaataagtttataaaggagattttatcatcatcacctttattttatggatgagcaaattaaggcagacctgagtcagacctaggtgtgtatcacttcagagcccatgttcttactaagttagtgtcaccatgatctctatcatgttgttaataccccttccatgaaaacattatcagggtaatacaactactgctacatcctctaataggaaatctactccttgggctagtagtgggttccttataccttctgacagttgcagcttctgattattggatagatcttcagaaaattcagattcatcctctgtggaccacactcccatccaggtgtggatcctgtgtaatttatcacttcatttctgtaaaatgtatttaccaactgctatgtgctaaggatactgatgtgactgtaacttagtttctgctcttaaggatctcatgatctagaccatgagacatgttaaagtactctgatagcagtactgtaatcaaatatgtataatctatagttgaagtaccaaatcagccatatctagaaacaatggcaaagaagtgtggcttacaagtagagaaatttgttaggtagacttaggagaaatgtgggaaaagtcctaaaaatagatttatttaatgatttttaaattagtttatttctattttttaatttaaaaaattctgtgggcatctgtatacgtaaagtaaaaactttaaggggttgtttccttcaatagatacccaaaggtagaattattaagtcaaaagatatgagccttttaaagagttttgatacatattgccaggttgcattcctaaaaagttatgcaaaattttatacagtcaccaacataaatgagcatgcttagtttgctatatcatactgagtgttgcattgtactcacagtcattcatgactcccctgatagtttctttgagtaacttttcttttcactttcttcttattatcccaaggtatcttctatcataaaaccaggtcagtcattagtagcaagttaccaacaattattacctttctggccaggcacagtggctcatgcctttaatcccagcacttcgggaggccaaggtgagagaactgcttgagcacgggagtttgagaccagcttgggcaacagaataaaccctggctttatataaaaattttttaaaaattacccaggcatggtggcatgtgtctgtggtcccaactacatgggaggctgagacggtaggatcacctgagcccaggaaatctaggctgcagtgagccacatttgcaccactgtactccagcctaggtgacagagcaaaaccaaaaaaaaaaaaaaaaaagaaaaagaatcattacttttctcttaactattcctaacatcaactggcttttagtatacatctaaccccctccctgtcgtcccagtctccctttcaaaatccagctttaaaatattacagtgcattttgaatgtcttgttataggtgtttgttagacacttattatatagagacttttatatttaagctttatacaagtgtgattttagctgagtgagcccaggaattagaagacctgaattcaaatctgagttctatttttttgtgtcatataaccttctgagcttcagatttctcctcttaaaatgggaataacactgcgtacttcacagggtataatgcttcgattaaatactgtgtagttacctgattcagtgcttggcacgtaatagattcacaactgtttgctaattctaaattaggcaggcagagcatagaagtctgattaggaagattcattgctaggtagcaattagaaaaaaaatcacatggtagtgaattaaagcctaccaaatgttacagagatgaatataaacttgtattacatataactgcagagagatatagtttataggaaaaaaacgtgtaaagagtactgattctttggaagttttctctgaaagtgagggttgagtcagcacaatttgaatgaatattgttgaatggggaattgctattaagttagatttggttgcctctaggaaaagagacttagggccatgtaaagatgatatttggcaatgctggtaaactggttaattgccagaaagtcttgttgtttggtggggtttttgactggatgtaataaagaatctctctcataaggcttttggtggagaatgtagtaagacacaagtcctgttgaggaatattgttcttgctagtgtgtgtaggcatggaaagctggtatagtgaggaagacttgggtggttgaggacctatgctaaacaggaggtgaccggaagaaatggtaaaagaacttagcaccatgcctggctgtgaacaaggggagtccaagaaaactaagtgtccaaaataacatataagtttataatcttagagctagagaaaaattaggaaatagtggattattatgtttttaattgaagtgtaacatacatacagaaaactatacaaagcaaatgtatggctccaagaattatcaaatgaacaaatgtgtaaccagcaccccagtaaaaaaaaaaaagtatttgtcagcaccccagaaacccatatcattttccctcacgatcatagctcctgtttcccacaaggtaacagcgatgctaacttctggtattacagtttagttttacctgtttttttattttatataaactagatggtatgttgctggcttcttttcattcaacattgtatttgtgagaaccatccatatttttacatgttgtggctcttcattttctttgctgtgtagtagttaattgtatgaatatatcacaaatatttattaagtccactaacccaaatagtagttggatatttgggttgttttcaatttggggctattataggtgatgctgtagtgaacatttctgtacgtgtcttttagtgccctggtacatgcttatcttagtttgctcaggctgctataacaaaataccataaactgggtggctcataaacagaaatttatttctcaggtttctggatgatgggaagtccaagataaaggtaccagcatggtcaggttctggtgaaggccctcctcctggttgtagactgctgatttctcctcacatggtgaaaggagcaatcaagctcccttaggccttttttataaagtttccattcctgagtgtttcaccctcatgacctaatcacctcccaaaggtcttacctcttaataccgtcaccttggaggttaggatttcagcatatgaattttgaggagacataaacattcaaaccacagcaatgtttttctattgggtttacacataaagtttgggattgcttggtcgtagggtattcttgtgttcaatttcagcatattgtttacaaatagttttccaaagttattccaagttatattccagtatgttatagaactttccattgccccacatttttaccaacgcttggcattgtcagacttcttaatttgtaaccattttggtaggtgtgtagtgttaccaaattgtagtttagatttctttttccttgacttaatgaaggcaagttcatgtttactgaccatttggatatcctcttttgtgagttactggctgagtatcttgtcagggtttttttctgagttgtctgtctttttcttacttgaaaatatcttctcccaatttgtgcctttcttctttattctttttttttttttttgagacagagttgtcacccaggctggagtgcagtggtgtgatcttggctcactgcaacctccacctcccaggttcaagcagttctcatgcctcagcctcctaagtagctggaattacaggcacattccatcatacccagctatttttgtatttttagtagagatggggtttcaccatgttgcccaggctagtctcaaacccctgacctcaagtaatctgccctcctcggcctcctaaagtgattggaatacaggcatgagctgccatgccagcccttctttactctcttaatagtgatttttggtgaataaaaagttattttaatgtagttcagtttatctattatgggtagtattatcgtgtcctgtttaagaaatctttccctatcccaagataatgaagctattcctcttgtactaccttctagaaactttattgttctatatgtaatatgaagtaaagatcaaatttagactctatactttatttggattcactagcttttctaccaatgtgctttttctgttctaagatctaatccaggataccacattgcatttagacactctaccttttgaaactttattttggtccaagattttaagcttgtcactagtaatactagattatcatacatcactgcatgtcccacttctgctcattcaagggccttacgttgctgtctgtttgaactagcttcttggtaccttgatctggaaataatcttctcttcctctgcatttctatagattttctttttctttccctctctcatgctttattggagtacttttgctgatttgtctgtcctttctatgtgatagataaaatcaggcctggtacatgtttggctaagtgagacctgagccctacatgaaactaagtcagatcctcttaagtgtagtctacactgttttgttaagatgataaggtgacactgggttgatgacttgatccaacctaacgtggttggagaattaaaactatagaattaagttagcctagttgttttcaatcattctgcttcacaagaagttaaaagactagaggtatttgttgaatcctcactcattgtctctctcagcttcacagattgatactgtgctcctacagttgtaactccaagaaacacatttgtctttttagtacttacagctgtgaagctaaaggcaaatttgaataatttctttaaatgagtgtatttaaaacattgacttttctatgaatgatctcgtattttctgctctgtttatgcgtttatattttacaacatacagattatgtcttaggtctccttaattatacctccaaaccgctagtaagtagcaggtgcaaaattgaggaattgagggaagaactttgaatgcatgttatatgggaattgtatacttatacaatatgtagaagtagcagttatttatatagcaagctttgtttatttttttaagagaagattgcctccagatgaataagcagtaaatctttcatttatgtgaagtaagttatgttttttaaaactgtcgaatagtttgttgtttgaacataattctataagatattatataggatagtattctaagagaaataaaagcatattttcagtaaaagacttgtacacagatgtttatagcagtcttactcatactagcaagaaatggaagcaacccaaatgcccatcttctggtgactagttataaaattatgatatattcaaacaatggactaccactgaacaatgaatagcaatgaactactgataaatgcaataacatggatgaatttctaaaacatgatgctaagtgaaagaagtcagataggaagagtatatactgtgtacttgctgttatttgaaattgcacaggaaaaaccaaccaacagtgtaataagattagtggttgcctaggaccagggtgggttgattgcttgactgacaaggggcacagggaactttggacgaggggttggtagaaatgttctatatcttgattattgtggttacacaggtatatacatttatcaaaactcatcacttaagatagatgcatttcattatacttaacttatacctcaaaagaagttaccttaaaagtttaagactgggcacagtaacccatcagcatttggggaagacccggtgagaggatcacttgagcccaggagttcaagataagcctgggcaacatagggagaccccatgtctacaaaaaaataaaaactaaacttaaaaaaggttaaaaagataaaaaacagtttgtgacttagaaaactgatgctaagagaaaaagggtctgagatcacaggttgaaacagagggatatatgggaccaaaagcaatgaatttggtcagggcagacctaattgcaatgataaactttgagactttcacatatgattaaacaaattgtgtaatctgatagtaaagccttttgtattgagtatgaaaattgaaactataatttaattcttttaaaaattatccattatatacaaggagaaatcctgtaaaagtctgaaggaaagcaagcacaactggagtctaactggttgttgaagtgctattagatctagttctgggaagttatgtggttatgtagagctatagagtttttggaagttatgtagttatgtcccaaggctttgtcctctggcattgaggaaaactttagtacttgttttaaattgatagtttttaatgtagtcattatgtatatgtatatatacatgctgctctaaagacacatgcacacatatgtttattgtggcactattcacaatagcaaagacttggaaccaacccaaatgtccatcaatgatagaatggattaagaaaatgtggcacatatacaccatggaatactatgcagccataaaaaaggacaagttcatgtcctttgtagggacatggatgaagctggaaaccatcattctcagcaaactatcgcaaggacagaaaaccaaacactgcatgttctcacttataggtgggaattgaacaatgagaacacttggacacagggtggggaacatcacacaatcacacactggggcctgtcgtggggtagggggagaggggagggatagcattaggagatatacctaatgtaaaggacgagttaatgggtgcagcacaccaacatggcacatgtatacatatgtaacaaactggcacgttgtgcacatgtaccctagaacttcaagtataattaaaaaaaagaaaaaagaaaaatctgggatggctggctttagtttatactcagctgtgttacattaactctctcaaaacaaaatgcggtagataactaggtcaataaatgtgatcattagttaaaatgtgaaaatgataaaattttctagaaaaataaataccaaaatcaactcaaaaagatctagataacctatattcattcgagacagtgaattagtaatccgaaatcctcctttctccctcttttccctaccagagtatactaaaacctagaaagtttgctgcaaagtttcactgtgccttcacagaacagattatccctgtattgtacagcttatttcaggcaatagaaaaagagaaaactaaataactattttatgagagtgatagcaaaagtggacatgaacaataccaaaaaaaattttttaagggaaattactgtctcagtgaatacagtgaaaaaatactaaatgaatagaattttgtagtgtgtacatattaatgtaattctctgtattaaaggattaaaagattaaaggaacaaaaacactatgattgttttaatagatgacattaacattttttgataaattttataattaaccaaaaggagagagacctcttagcaaatttggattaaaaggaatctaggctgggcatggtggctcacatctgtaatctcaacatttagggaggccgaggcaggtggatcacttgaggcaggaggtcaagaccagactggccaacatggtgataccccaactctactaaaaatagaaaaattagccaggtgtggtggtgtgcgcctgtaatcccagccactccagaggctgaggcaggagaattgcttgaacccgagaggtggaggttgcagtgagctgaggtcgcaccactgtactccagcctgggtgacaaagcgagactgtctcaaacaaacaaacaaaaaaatctgaaatttcttttacctaataaagagaatataacaaaaacctagagtgagcaatcatgtttaatgataaaactttagaagcccttccattaaaatcagaaaaacgttaggaatgtgtgctagccctgcttctattaaacaatatgctagagggcttaggcactggaataacatgagaagaaattaaaagttaaaagaagagaaaaaattggtagtgagaataaaccatttatgttttgtaggaaattcttgtcaagaatggctctactgctccaattctagagttaatgtaaaacttaagtttaaaaaagccaggttcgggaacaggcaacctacaaaatgggagaaaattttcgcaacctactcatctgacaaagggctaatatccacaatctacaatgaactcaaacaaatttacaagaaaaaaacaaacaaccccatcaaaaagtgggtgaaggacatgaacagacacttctcaaaaaaagacatttatgcagccaaaaaacacatgaaaaaatgctcatcatcactggccatcagagaaatgcaaatcaaaaccacaatgagataccatctcacaccagttagaatggcaatcattaaaaagtcaggaaacaacaggtgctggagaggatgtggagaaataggaacacttttacactgttggtgggactgtaaactagttcaaccattgtggaagtcagtgtggcgactcctcagggatctagaactggaaataccatttgacccagccatcccattactgggtatatacccaaaggactataaatcatgctgctataaagacacatgcacccgtatgtttattgcggcattattcacaatagcaaagacttggaaccaacccaaatgtccaacaatgatagactggattaagaaaatgtggcacatatacaccatggaatactatgcagccataaaaaaggatgagttcatgtcctttgtagggacatggatgaaactggaaatcatcattctcagtaaactatcgcaagaacaaaaaaccaaacaccgcgtattctcactcataggtgggaactgaacaatgagatcacatggacacaggaaggggaatatcacactctggggactgttgtggggtggtgggaggcgggagggatagcatcgggagatatacctaatgctagatgacgagttagtgggtgcagtgcaccagcatggcacatgtatacatatgtaactaacctgcacaatgtgcacatgtaccctaaaacttaaaagtataataaaaaaaaaatatatatatataaaaataaaaaataaaataaataaaaaagccaggttcagttatagttgatgttgtctctatctctctgagcctagtaataataaaacactgttggttctgggatagtggaagaacttccttttcatttagcagttatattcataggttgtgcttaaactgattgtaattaaactgatgaaattatccaactaccaccaagtagttgtatagattttaaggatatctgtgagggaaaaaaatggtctattccaattattgaactactgttttatgtaaaaataatatgaaataaaagtggtatgaaatagaaaatggatggaaggatttttttgtggtaataatatctcttaaacttatattctgatttagggttgccttagtctgcatttaaacctgttcacatgctggatccaatcccagggccttaaagtacaaactgcttagccgaacttagtcttagctttaaaagccgaggtaacattgcagacccatggtgtattttagtcttagtcattatttactggtagcctggacagagtgcatggcatgtgctgttctgtgtcattcactctccttcacttcctccctacaatcctattttataatcagtttttacattttattgtttgtttatctttcctcttaggaagctgggattttctttttgctgaatggattgaaaaataattggggaaaaggaaaccacaaagagtttagagaggtttctgttaagtacaaaaattaacatttgagttaaattgtcttcgaattattttcacattatttatatatttaaaatgttttggctttgctcataaattcttcattgttcaaaacattgcttttgtaaaatttgtagtattccctttcaccttatctatcctgtatctattattatttttccctctttcagctttttgatgagaccacaaaggataatacttagaggagtttcctggcctgtattacaagatagaccatgagttctgcctcaattcaacttcattgtgtcaacttgataggataagacaggtggacattctgctaaccagcatctgattagagagggtggaggctggtgatggattgttaggtgtgatgacaaaataagcaattccgttaacatgagtgtgcagagtaaaattgggaccagcagatggtggggctaagctgtatcttatttctcagctatgagattttccgtggccgccttttcacagtagccagctgggattgtccattaactgggtttgagtaaaagggagttgttgctttctttagaatttgttcagcctctccttttcatgtatggctttatgttcatttggtagtaaaacacgatattcaaaggcagaatatatgagaactgaccttttcttggagaacatcccagttagatcccatttccacaatatgattacactttgaaatctggcttttccctgttctttctttaatcctctgatattttaaattcctgtaatctctgctattgccactttaaacctcattactgaaagttcttcccacactgaaacacttctcagaaaaaaaatgcagaatatagagcagagctataatataaacttaaacagacctgctagttttagctttcttttctagtatacataatttagtttacttgatccaaaggatctttaagaaacatgttttggtttaatttctgtttgttttgtttttttttttgagacagggtctcactgtgtcacccgggctggagtgcagtggcgtgatcttggctcactgcaacctccacctccagggttcaagtgattctcctgcctcagcctcctgagtagctgggacgacaggagtgtgccaccacacccagctaatttctttgtatttttagtagagatggggtttcgtcatgttggccgggctggtctcgaacttctggcctcaagtgatctacctgcctcagcctcccaaagagctgggattacaggcgggagccaccacgaccggcctggtttaatttctaaaacttacctactaatcgacttagttctgcaataaatatagttacaatcattataactagtattccttgggctggtttaaagatgttctttagcatttgagatgaaaggcagaaaccacaggtaggatcatgtaagctatggaaccaaaggaaaagcctggaaatgcaacttggagtcctgcttactctgtatccttggaaaatccagattgtgaaagaaaagaaaaagatcattttcatccatcttttgacagctttctactttgacacttctttcctctacagttccaacagaaagcccaaggctgactttgatttgcctgacttgggtatgttcccatccctgcctcaatcattaacttactggcctgagtcttagtgatggggtcagcctctcctcaatcctatgagcttggaacaggaaaggaaaattggagaagaggaaagggattctggacagtcaaaaataattaaatatccactctcttcccaaagctgtgtaatgggagagcactgtccttcagccaataatgcactagcagctagattccttagctagaccttcttccactgttgaagcctaatccctctgttttgctgcagatacctgtttccgaagtttacactgtgctggactgagtttgtagacatgaaggtccatgtaccctgtgaaaccctcgaatacattgaagccaactatggtaagacctggaagattcctgtaaagacgtgggactggaagcgctctcctcccaatgtgcaacccaatggaatctggcctatttctgagtgggatgaggttatccagttatattgagatagtaggttgaaatgggagaatttctcttttggaaaaaaaggtagataactgtttaaaaaatacatgtctatttgtcaaacataagtgggaaccaaagaaaaaatgtgacaagtttgaagacacagaaagagtcatctgatgtaattctctcacttagtactgaggaattttcatgtgccacatacaatgctaggttacagtggagaagcctagatgaatgagacaaatacctacttcttttattcctccttttggtaaacaactcaattttcctttgagggaaccctcccccaccctttgaagagttcaagttctgtacaggtttttaaaacgtgaagtaatgtttgaactggaagatgagctcaccaggcaaagctaaggaaggatatactagttgaaaagaataacccactcctcttctgggcatttaagctggtatgttagtgctacttttaagattgtggagtctgagttaatattcaagtgatcagactttgagtgacatcaagaaaagatgatatcaggttcatttttcaactaatcttatgtggaattgaattagagaacaaggcattattcttttagggaaggtgagagcttatttgtatcagagcttattacttgtcaggataagtaaatttctgtacatgtactgttttcatatgtgaagtgagaagaaactttatgcttgtttaatgcttaaatttccatccattgtgagaatattttcactgacctctgatggcacttgttgacaaatcattcaagtgagaccatgttactagacatgatcttgaaagaggccatgatttcacaaaactcatttttattttattctcagacagtctgttaggtaaaaatatgagaaattcatgtacattttatattttctgaatttataatctgtgcactcccaattttaatgacactaaaatattaatagaattttttaaatatactctaatttttaaaacatactctttattatcttcatttatcaattacagcttcgtatctctaatttatggtctatataccaatttaaatggcatgtaaacctgcctgtttcttctcctcttctaatatatcagatctccaaaatggaagctaaatggtggacttgacaactgttcaccctacctcagatcatagagtttgtaaagtttgtgtccctccccagtttttcagtctgttgaatgtcgatggggcaagaactcagacttctactttaccaagtaccacacactctggaatgctttagtttccttttcccctcaagatgtctgagtcagctaggatgctgtttaccccatctctctcttatatcacttgaatgatatattgtaagtgagaggtaaaggaaaatgtaggcacaataagcactgctatttttctctttgtctaggaaaggaagctgaatcttatatcttatctatgctatttaggactactttctggagcttggcagattttcctctgacaccagagaacaatagtagtctcaagaatggaaacctgaatgtctgagggaatgggctggtagactttttcgaaaacaaattagagaaagtaacttacaaccacccattccggatttgtaaagcaacatgaaaacctttgataaatgataaccaacagtcttctgtcctaatttgcattctcaatgcagaattattgggtctttcataaataacatgagtggtttctggagacatttaagattgtcagcaaacttgtcccaaaatggcacatcatcataatccattttctctttgctagaaaatcagcccatagagtgcattcccaaattctaaatagctgaccctaaattcatttttcatgcttaaaaataatagaacaaataataatactatttttgggcaaaatccaccctacttgatgaggaccatttgcttgtgctcagtatttagaaatgcatacactccacatttctccccatttccaattgggactcccattctttgccaggagatcttacccatcccttttcagattaatcttttatcctttcctgaagtacaaagtcttaagagtgtctgaaatccaagacatcttggcccaattgacacaggttctatattcttccctacatagaccactggctgctgaaatacttttcttgtcttctggtttcacaggcttcagctcatgggttccaccctaacttggggaaacaaaagccttctctagaatctgaaggccaggcttacctctgattctgattcatccatacttcatcttatgtattttaacagctgggttctgtggagtgtccagagaccttgggttaggtatatccatcttcagtacctcattggatcacttttctttcatcacttgagtattctagcagtcattctcctaatctgaccactttcaggtttagtttacctggcttacctggggaagttgacaacttgttggtagttaggcacccatgaatgtctccagagacatcctgagaggcaagattcctcttaattgataaccaggacaaccaggtagtcacccagtcctctctaagcagggagcacttgtccttctctcctctgctgcagctactgatatctggcccctggaataaaaccatagttcctaaaattgagcatccctaagagtagctgcttggtgggacagctgatttctttgattccctagctgcaaaacctgaaattgaccactaggtgacagaatgtttgccagtatccccacaaaacaagttaaaacttaagtgaaaatcattctgcttttgaatcttaaaagctagaaaaaccataatgtaatattctttttaaaccctcttattttataactaaataaataatcacagaaaagaatgatctgaacaagaacagctgaggctaaaacccaagactgccgtgactcctagtccaatgtctgtttcgcatcacaacacagtatctttaacagtgcttgagatgcttaacagagaaggcatccagtgcttcattgaggctaagtctcagggtgtttctgccgcttagtatctttttgttcagattgagaacctaaggcgacagagaggtcaaggggaagtattttctagttcagaattcagaattcttaggcaaccttcatacctttatctggaaaatgccttctctccagacaataagacagttcacatctggagacatcagcctttggtacctaattctctaagctcaagatgcatcccattgccactttaccattctatttcccaagggaaccatcagcaccaacctgctaaatgcctgtatttgaagtctctccccttcctgaagtgaccttttatgaggctctttccttcctaagggacctttccctggtagtagtggtctcattcacaaaaaagaataatagatgtaactggagtcactttgcagttttcaagattttttttttatctgcttggctggaaaggagactagagtatctagtttttagtatttaaactacttttaattatttatattgatactctctgataaatgcaggtagttaagaatagattgtactcattcctttttgagtttgtgacctcaaaccattgtttttattcttacacgactacagtacttcaaatggcacatagataggcaggatattacataggtaagcaggaatttatacattgggtaccagagctaaatctggaaaacacatttggaatgagcttccacacttcagtctaaaatctcacccaaacttatggctacatatttttctaagtttcccccctagtttcactttctggaaagtgaacagttttttaaatcctaaatgttataaatccttaggagaaatattccctcaaaacctagtcaagaaagtgccacattcccaccttctaacaggtaattattagttgtaatagctttaatgcatggaaaaacttcagttactgaccagtcaagagaatttctcaagaaaaatcccagcaacgttccctctttcctccttgtcttccactatcattaagacctgggctagatcacctctaacatctcactcagggaaggcaatgtgttgccataaaaagaccacaagcttttgagttaggcctgaatttgaatttcagcttaatcatgtgggatttatggtgggggccctttcagtctcaatttccacattagtgaactggggaaatgatacatacttctaagggtttttagggggattaaatgaagtatacagttcttagcctcaggcctaggattaagtaagtactcaagaaatgtgcaattttctagttccatgtttcttttctaatcttcaaatggaattatagaaaccatgggtcagaacatattcctttactcaaaagattgcatgactgaatttgcttaagaaaaaaaaaattgtgtctctccctctccctctccctctccctctccctctccctctccctctccctctccctctccctctccctctccctctccctctccctctccctctccctctccctctccctctccctctccctctccctctccctctccctctccctctccctctccctctccctctccctctccctctccctctccctctccctctccctctccctctccctctccctccactgtctccctctccctctccctctccctccacagtctccttccacggtctccctctgatgccgagccaaggctggacggtgctgctgccatctcggctcactgcagcctccctgcctgattctcctgcctcagcctgctacgcctcactggttttcgttttttttttggtggagacggggttttgctgtgttggccgggctggtctccagctcctagccacgagtgatccgccagcctcggcctcccggggtgccgggattgcggacggagtctcattcactcagtgctcagtggtgcccaggctggagtgcagtggcgtgatctcggctcgctacagcctccacctcccagccgcctgccttggccccccaaagtgccgagattgcagcctctgcccagccgccaccccgtctgggaagtgaggagcgtctctgcttggccacccatcgtctgggatatgaggagcctctctgcctggctgcccagtctggaaagtgaggagcgtctctgcccggccgccatcccatctaggaagcgaggagcgcctcttccccgccgccttcccatctaggaagtgaggagcgtctctgcccggccgcccatcgtctgagatgtggggagcacctctgccccgccgccctgtctgggatgtgaggagcgcctctgctggccgcaaccctgtctgggaggtgaggagcgtctctgcccggccgccccgtctgagaagtgaggaaaccctctgcctggcaaccgccccgtctgagaagtgaggagcccctccgtccggcagccaccccgtctgggaagtgaggagcgtctccgcccggcagccaccccgtccgggagggaggtggggggggtcggccccccgcccggccagccgccccgtccgggaggtgaggggcgcctctgcccggccgcccctactgggaagtgaggagcccctctgcctggccagtcgccccgtccaggagggaggtgggggggtcagccccccgcccggccagccgcccagtccgggaggtgaggggcgcctctgcccggccgcccctactgggaagtgaggagcccctctgcccggccagccgccccgtccaggaggggggagggggggtcagccccctgcccggccagccgccccgtccgggagggaggtggtgggggtcagccccccgcccggccagccgccccgtccgggaggtgaggggtgcctctgcccggccgcccctactgggaagtgaggagcccctctgcccggccagccgccccgtctgggagggaggtgggggggtcagccccccgcccggccggccgccccgtccgggaggtgaggggcgcctctgcccggccgcccctactgggaagtgaggacccctctgcccagccagccgccccgtccgggagggaggtgggggggtcagccccccgcccggccagccgcccagtccgggagggaggtggggggatcagccccccgcccggccagccgccccgtccgggagggaggtgggggggtcagccccccgtccggccagccgccccatccgggagggaggtggggggtcagccccccgcctggccagccgccccgtctgggagggaggtggggggatcagccccccgcctggccagccgccccgtccgggaggtgaggggcgcctctgcccggccgcccctactgggaagtgaggagcccctctgcccggccagccgccccatccgggagggaggtgggggggtcagccccccgcctggccagccgccccatccgggagggaggtgggggggtcagccccccgcccggccagccgccccgtccgggagggaggtggggggggtcagccccccgcccgaccagccgccccgtccgggagggaggtggggggatcagccccccgcctggccagccgccccgtccgggaggtgaggggcgcctctgcccggccgcccctactgggaagtgaggagcccctctgcccggccagccgccccgtccgggagggaggcgggcggggggggtcggccagccgccctgtccgggagggaggtgggggggtcagccccccgcccggccggccgccccgtccgggaggtgaggggcgcctctgcccggccgcccctactgggaagtgaggagcccctctgcctggccagccgccctgtccgggaggatggtgggggggtcagccccccgcccggccagccgccccatccgggaggtgaggggcgcttctgcccagccgcccctactgggaagtgaggagcccctctgcccggccacgaccccgtctgggaggtgtgcccagcggctcattggggatgggccatgatgacaatggcggttttgtggaatagaaaggcgggaagggtggggaaaaaattgagaaatcagatggttgccgggtctgtgtggatagaagtagacatgggagacttttcattttgttctgtactaagaaaaattcttctgccttgggatcctgttgatctgtgaccttatccccaaccctgtgctctctgaaacatgtgctgtgtccactcagggttaaatggattaagggcggtgcaagatgtgctttgttaaacagatgcttgaaggcagcatgctggttaagagtcatcaccactccctaatcttaagtacccagggacacaaacactgcggaaggccacagggtcctctgcctaggaaaaccagagacctttgttcacttgtttatctgctgaccttccctccactattgtcctatgaccctgccaaatccccctctgcgagaaacacccaagaatgatcaataaaaaaaaaaaaaaaaaaaaaaaaatcaagtcattaatacaattatacattaattatattacattaatacaatatatggtttgtgaattcagagacattaccagtttgcctccttctctcaatagaacttgtattttcattttcttggttaagcagttgtctcctaatattatcccatatgctacctagtttgctggtcccaagcagtttactgtacttcactagatttggtacctgctctcccctggacttctttttcaatattctagcctttcctagatgtaaatctttacctccttgttagtgaaattagatataagccatgatttggagagggaagaaatctggaatacttaatttcatttaattatctatgctgatgaatgcctgtatcattgttaataaaggagaattgaaaatactcatttctactttctgccctcaaatttctgtttctatctcaactaggcaagaatcagcagggtgcatgatgccattttaagctgcttcacatcagactgaaatcctaattacagttcataagtgaaacagactaattcaatggcaataccttttgtataggtcctgtgcttaaaggaggcaagtataaattttctaataagaaatccctgcttcttttgggtgcagtggctcacacctgtaataccagcagtttgagaagctaaggcaggtggatcacttgaggccaggagttcgagaccagcctggccaacatagtgaaaccccgtctcttctaaaaatacaaaaaaattagctgggcatggtggtgcacgcctatagtcccagctacacaggaggctgaggcaggagaatcacttgaacccgggaagcagagtctgcagtgagccaagatcgcggcattgcacttcatcctgggcgatagagcaagactctgtctcagaaaaaaaaaaaaaggaaagaaagaaatctctgcttccgtactatcaaaacttctaccctagaataccccctggcaccttctaacccaacctaatacagagattttgtagggacccattaacaagctcctatataattataagcagctctcacagtagggttgaaagagaatataaggaaaattagaagtactgtatttttgctattggaaatgaaatattgtttcatgcacctttgaaaaaaataacaggattttacagccttctgatgattcattcaaagcatggggaatagttcatatgtttgttaaatgaaaatcttatgtagctatttgtgtgtccctcccacttcataactacaaaaacatatatatgaatttctaaacaaagtgatattttaaagatgaattgattcaatgtgtacttaccagtttactgtgtggttttatcttcaggtacagatagtttgtggtactacttgaaaatacctttaatattattttcatcagaatttgtaatatataatccagtttgggatgatgaataaaatttttctaatctcttgagatatcttgtatttatttttgagacttgcagtagaaataacagacactaacattcacagacaatctgataaaatagtaatcttgccaccagtacagtatttctaaaattcaactatggggaccctagtagtctgcacacatatacctgggtatccaaaagttctcagagataaaacctgccagccaaagaccaccaggaacacacctgtaatcaaacaaagttaggtttattagcttgttgtagtaagaggaaacagccaccatggggaatcataacatatttcagggagaaggaactagaaaggtcttttataggctttgagctgatgtcaaaattgttaaaagtaactgtggtggagtggaaataacacaggacatggagtaaaaagttctagtttgtctgaatccaacagtgccatgaccagtaggattcatttcaggtgtacatggctagttcagccttaaaacagtcaatgtaatgcactgtatcaacaaagtaaagaaaatcatatcaatagacacaaaaagagtctgacaaaatctaaccctcattcatgagaaaaactcagtaagttaaaaatagaagataattacctcaacttgatgaagaacatctaaaaccaacaaacaaaaacctgtatgttttaatagcaaaaaactgaatgtttttcctctaagattaggaacaaggcaaggatgtctgctttcatcactcttattcagcctaatactagaagtgctagtcactgaagtaaggcaaaaaataaataaataaataaataaataaaagacatgcagattgcaaagaaatttttaaaaacttttcatttgcagatgacatgattgtttacatagataataccaaggaatgtattttaaaacaagcaaacacctggagctaataagtgagttttagtgcagtcacagtatacaagatcaagaccaatacccccaaatcaattgcatttctatattctaacagcaaacatgagaacaaaaacacagtactatttaaagtcaccctgaagaaaatgaagtacttaggtataaaattaacaaattatatacaagatttgtatgttaaaaatgctgatgaaatcaaagacctcaataaatggagatgcataccatgttcatggattggaaaacaacacagtaaagatgtcagttctactcaacttgatcaataggtttaatgcaattcctatcaaaatctcagcaaggtttttaatagacatagacaaacttattttaaaatgtatgtgataagtttatttctctagaatatctcaagtaatctttataaggaaaaagtagcagaaagatttggtatcagaagacctaagttcattcttgcacttcaatagataccacatctgatcttataaggtagatgttatttccccttgttttgcagatgaggaagctgcaatttagaggtaacacagatcttaaatccttgttttctgacttgaaatccagtggctactcactctgccaattctacttaactgttgatctgaaaaaaaaaatttttttttaattattacttaaaaccagcctctgatactgaaagtgagaaggatcactctacccaatattaaggtttattatatagctatagtaattgttatgggctgaattgtgttcccttatatccctcaaaattcatatgtttcagtcctgacccctagtatctcagaatgtgactgtgtttggagatagagcctttaaacagctaattaaggtaaaatgaggtcatatgggtgattcccaattcactggtgactagagtccttagaagagcttaggacaaggagaggcacagaaggaggaccatgtagagacatagagagaagatggtcacctacaagccaaggagaggatccctcagaagaaaccagccctgccaacaccttagccttggacttctagtttcctgaattgtgagaaaatagatttctattgttgaaaccactcagctgtggtactttgttatagcagccctagcaatctaatgcagtagtcaagacagtatggtattggtaaaaggatacgcacatagatcagtgaaacaaaataaaccagaaattgacccatatgagtatgtccaactgattttttacaaaagtgcaaaagcaattcagtggaggaaagacagtctgtttttttttattttttcttttatagacagggtctcactgtgtcacccaggctggagtgctgtggcacaatcattgttcactatcacctcgagctccatgggctcaagcagtcctcccgcttcagcctcccaagtagccaggactacaggtgtatgccaccacaccccgctattattttattttattttgttgttgacacggagtctcattatgttgcctaggctgctctcaaactcctggccccaagctgtcctccacctaggcctcccaaagtgctgagattgcaggcatgagcctccacacccagccaagatagacctttcaacaaatggtgctagagcaattggacattcataggcaaaaacaaactcaacttgaatgaacctcacactttgtacaaaaatgtacttaaaatggatcacatgcttaaatgtaaaatataaaactgtaaacccttttgggaaaaaaataggagaaaatcttcatgatctagggttatgcaaagcattctttctttgacttgacacaaaaatcacaatgtataaaagaaaaatggataaattggacttcatcaaaattaaaaattgctgctctgcaaaagcccacatgtaggggctgaaaagtccagctacagactaggaggaaaatatttgcaaactgtgtatcttgacaaaggactagtacctggaatatataaagaacctgaacactcagcagttttttgaaaaattcaattagaaaatgggcaaagacatagacagacatttcattgaagaggatatacagatggctaagaagcacatgaaaaagatgttcaacatcattagccagggaaatgcaaattacaaccacatgagatatcattgcatacctattagaatggctaaaattaaaaataatgataacaccaaatctgctagttgtttcttttatgattttcttttttaatgtgtactgtgcaccgttgtttttactgtgattttactaaagagtgtccttaaacattttacaaacattcgtaataggtaacactcttcataataaaaaggaataaccttgtctgaatttttggaagacaggtttttaggtttttgtttttgcctttcctccaattctttgttgatttactttgtcattttaataaccctctttttatgatttattttctctttattattcctttgtgttcttcgagttttctttaattagatttatcagtaaagccctttagcagctagtactattgttcatagttctctgcaactttatcagtagggcttttacaacctaaaacttctaaattcaaattttttcttccgttaatctcaataatttggaggatgttttctagtgaattttgcaggaaagttaattgagtggccaatgttctgaaaatgctatactaccaaatgtctttcagatgacttagaagatgacagtctcatagttggagagtggaagagtttgctttggagcccaaactgggcaaccgtctaatccagccagatcctgcttagcagaaaaagcaaatttctggcatgtgacctcataaacaagggaaaagctctccttttaggatgatgtcttctcttaccatctatttccccatgtcttagtggaaggagccatctttttccccatgtcttagtggaagaccagagaattatctagagcatggtgtgatgctgcaaatgatgtatctgtagccactagccacatgactactgaatatttgaaatgtggcaagtgtaactgaataactaaatatttactctaattttaattaatttaaaactagtagctagcatattgcagatctatagggttttatgggatcagcaagggttttggatttgtcgactggaatccagagccctccacagcctagttcggtgatcttgggctagctattcaacttctgagttctgaattttttttcaactaatggggctaaattaatacctacctttaaaggttattaaaagaattgtaagaaattgtaagaaatctgcagtgtctggcacactgctcagtacatggtagatgtacagtacatggtagatggtcagtgaatgataactattgttaatattatgttcacatggttttacatctgcctttggcataaatcctatcagcttgtattttcctgataatctcatgtcacaatttttctgtaagattggtatttcagatccctcctgggtagaggccctatcctgagcactggtgttaagaagcgaccctggcctcaagagcacaggtacaaggcctgttctttggggagagagtatgtggggttaaaacataacacttaatggaattgagtctcaaggaccaggcttaggcaaagagacaaaagtcctagactttgtagatggctgtctgagcacccgagtctagaaaaagctccaggaaggaggacagggactgggtaatgaggttcagctgagtcttaggacttgtagaacagaaaatttgaataaatgaagaaagaaaacatttctgagtaagaggagtcagtaaattcacagaataggctttatgggacagtgaataagaccatctgccatatggataaatagtgaaagatacaactggaaaagtggtcaaggaacagactgcaggaaatgaggggactgaatattctgctatgaagtttggatatgagagagaaaagttttgaataggagcatcatgccttcaataaacacttctggcctggttactactcatcggatctgtcctaagggtgaggttcgacaaacattcaggaaaccccttcaaggatagagcagggatttaggagaattcagattcaccgagactgatcctagagaccctagaaccctgatagttgcagggacagaggatacaaacttagccagatgggcataggaccctagtggtttaagtaaggtcactcctaggaattatcagtcagtgctagacatgggcacaagcagtccagagtcaggaagcgcttgagaccaagtgagcaggggacagtttggtgatggtctgggaagtggagctcaagagcagcattgcaagccacagaaagggagtgtgataggacaaggcagggtcttatccagagggttccagggaattagaataggcctttgagagccatgacaaaagctcattttgatgaattgggccaggagagccagtgagattctaggctgtggagaagacatgaaggcaatttttggaagacagcagaggaatggagaccaatggtcagtgctagacctgggcaccacaatacaggcaatgtgagggatgtgggaaagaggctggagccatttctatacctgtcgcttcagttagaaactaggacaggatagacttttcacatgatgatgccacagggcataactgaaagctagggagaacagaagccaggaagggagataagcttagtgaggattttaaattctgggtcttaacttagtcctcatctccctattggctgttcacctctggagactatgggctccaaggcgtaaaaagtaattgctctagttgtactaggagagtagtttgtgctaacaactgaccttctaccctacatttacctctacgagaaggcttgggactccagtggctttctggaccataataaaaacaaggccattttgtcttcactcttcctcgtttccacccagacagattctgctgcctggataagacagctcaggcagggaccgctggctgacgaggcctgggcaagcctataatcccagcagagagcacagggacaatgagtgggaggggagccagtcacaggttgtatcttattaaaccagtctgcatcagctacagtgtacgtctcagaaacagatctgaaaccccagctggtaacctagttagttcaggcagcgtgtaaagaaaccatatccccgccagctaaaaagatgcatgtgctcctgggtagtgcagaagtatctgttatgaaaagcaaaggtaacaacagttgtgggaaattaaggtttcctctgtgtgtttttttattggttgcatttgaggtgacatcctctaattttcctaagcacagtggggcctcctggaaacatctgctggatttgaggagtaaggggatgcttccctcatcctccgggtgtgtgtatttggtttgggatttgtcaggctgggtagctgagggctctgggcagcttgacctggcagatttcccccacttgcctgaaaagcagcctagggggcagaggcccctccccaactcagccctgcaccttcactctaagcgcctggagctggggccttttatttcaagtctggtccccagggagcagagtgggaaatgaggacagctgataagcctgacagtattgactttatggggagtattcaatgaatttactttctgcaagtaggctgcactcttatctgctgcccacagagcatctaaatcctcatctaggagacccatcgatgagtcacgtcccttacacaaagaccagagaataaagaaggaaaggggaattccatccacccctttcttttctccagtacctggtcctgcccaccccaacacctcccctcgctttccccactgcgtttgggtttattggctgaaaacagaagcactcgcagctccaggcctacggagtcaaggccaagccagcctggtcttgagaggtcgacagctgggcacacccagggctgtatgtccctctaactggtaactatgggaagctcacttgaagtagttgtgtgcaccgctttatgctgcaacagtcaacatttgctctggacagaaataccctcacggctttaacgccaggtgtcttggagataaaatgtgggtgtgtgggcgttaccaaggggtcctgggtctggggtgctggagagtggaagttacatgtaagagaaaggcctgatgcgcaagagaagtttttctttcccctctggcttctccctcatccagtcctgggctctgtttcaaatattagaaaaaaataaaagcttcttagcagcacagaaagtaagtaacttgaaggagagaggtgggagccagaatgctggattgggcagatgaaaggaaaaaactgaaagtgccctttggcagaaattagagtcatgtgtttaggttcaccatctagcttttagacagagttttttggtagtaaaaataaaatgaaatctctgtattgagtaactttggtttcattagatgacttagcaccattttttagtatttattccaaagcactaactttttatacattagctcactgaatcttcacaataacccatgagatgatatttctgagttatagctgagaaaactgagtctgggataagttaagtaacttgctcaggatgacaactataatagcatcaaagcaaggatgcaaacaccagccagtctgcctccaaagccaagtcaaaggtcttctcttagctgccacactaaactgcctgctatttggcatttttcaatatcttatctcagtccatggccaatcaatgagtatttattattcccacgttattggaaacaggcttagcaggataccactacctgtccagggccacaaaaccagtgtatatcagagactctggtccacagagtctagcatctctcctaaaggtctcgccctgctggtgcattgcccactgctcaggcagagatgtgggccacatcagtgcgtttctcccttccaggtgccctggtttcctgtgtcacctgctttcacctgctgctacttgcttgataattttcttagttgagggaggttggaatgagggaggcaggaagagcctgggaggatgtgagctgttcactaagttgctctgtgggccctgtgaatggagtagtatgaacatccatgagaatctgcagcttctgcaggctctggaaagatgcctgtctaaaaaccgctagtaaaactgagtcagccatatgcttgtttctttaagtatatgttttagtatttgacttctttgggagaaatacattttttgtttaggataacttgttatgtaactttataattaatatttataattgttcatattgaataagaaaaccttggtgaaatgcctagcatgacacttggcacttaaggttgaataattggggcagaggattaagttcctgggccagagttgatgcttaatgtcaacccctcctcaggtcaagccatcatctcctcttgcctgcattgctttcacggcatcctaactagtccccccaccccacctcttctcttgcccctctccatgtagcagacagaatattctctccttcttaaaaaacaaccaggttgggcgccgtggctcacgcctgtaatcccagcactttgggaggccgaggcgggcagatcacgaggtcaggagatcgagaccatcctgactaacacggtgaaaacccatctctactaaaaatacaaaaaattagccgggcgtggtggcgggcgcctgtagtcccagctactcgggaggctgaggcaggagaatggtgtgaacctgggaggtggagcttgcagtgagccaagatcgcaccactgcactccagcctgggtgacagagtgagactccatcttaaaaaaaaaaaaaaaaaaaaaaaccattctatggccttggaaacatttacctcacagaagcaagctatgtgtctgctgacagaaggcagggcaggctggaggcagctgtctgaagaaataagagctttcttgcattcattcaacaaatatctgatcaagcagcttttatgggcagtgagcacaattcctggggtctagtgatgaaggaaactaagtctttgtcctcatgaagtttataatgtagcaagtaaactagaatgagatttgttttgcagaattcaacatgaaggtggggtctcctttaaagaaaaaaaagagagagttaaaataattgaaatttatcaaaaagagtttcttatgaccaagagtcactcccacgcaccccaaattaagtataaagaatgggcacagtttactttggaaaatgcaaatttaaaagcaggggttgtaatattaatataataaaatgaaattcatggtaaaaagcaagatttttatattgatataggctacaatcctctaagtcaataaaaaaacttccttgagtctttatgcttcaaaagcaatgcagcaaaaaatgtaaagatctaaagcaaacactcccggaaaaacaaaaagaacagaaacaaaatagtaaagggagattttcacacagtgctctcttgaatagatcaaatagacaaaaacttccaagaatacagatttatttaatggatgtgtaaaaagacattttaccattcaaacagagaatatacctccttttctagtacctgtgaaacatttataaaagttgaatatatgttttatcaaagagaaaattctcaataaatatcccaaagcaaaaaacatacagggcatatatttcactatactgcaataaaattagaaactaatagcaaatggttgccaaaaaaatacaacaacaagaaaatttaaaaacactttataaaagaaaaataagcaacagacattagaaaccaatgacaatgatactacaaatggaaacaggatatccccaaaggtctatcagaagaaagttcacagcccggagtgcttttcttactaaacaagaaagagtaaaaataaataagcattcaatccaagagtgatagagtggagaggaaataaacgtaaacaaaagaacagatttaataaagatatagtagaaagtgtatttgaaaatcataaaaatgataagcgaatcccagagctagttttttaggagcaataaaatgaacagacttttgcaacactgatcaagaagagagagagagaaatcataaacacataacatgaggcatgagaaaggggattaaaaaaatagagatgttaaaaagtaactgaataactgtatataacactctactaatgaatctgaaaaggtccaaatttatatgtcaaagtaccaacattaaggagagagagaacaggggaaggaacaaaacctacctagaaggatttactagtaaattgtattaaatatcaagaaccagctaactcatctgtttaataaattaatggtggatggaaaaagtgatgaataaatgactggataaatggagagatggatggatgaataggggcctcgatacatagaattggagattggtaaaggggctaaggatggaggagggaagaagagagttttaagagtggctaaggctgatgcttgacctccagccaaaacaatcttggcccacacccacttggcctggcagaaatcccttccaaaagtcccaggtttgggccctggcggtggctgactcctgtaatcccaacactttgggaagccaagtccggaggattgtttgaccccaagagttcaagatcagcttgggcaagatggcgagatcccgtctctacttttatgaataaaataaaaaacaaaaatcccaggtttggtctttcctgaaactgacaacccctgcatacaggactagaaggccagtattcacaggctaatccagacagatcaattaaaccaggagaaccagaaagcctgacagtgcccaagctctcctagtgacctgcccttccctccccagccctctgtttcctccccaggagctcgcaggtgcagtctctccagggggcagtgagagccatgaatagtaagggttttagctcaagcacacagaggcgtttagctgcccaaatctaatcccccaataatcggcttatgtaaattcctacttcaaccccttcccctgcaggtcctagccccaaaattctctacattgggagactggcatgggagaagacccatcactctgaaggatcactgctagtgaaatgatgcgccaaagattgtttcccctgcttctgaaagtataaaaccaacaataacatttaagaatgttttgaaaagaaaaaaccatcaaccctggtcccaggatgtcaacacaatcgggctcctttctctgtagcccttgtcctttctctgagtccttgtccactcgcacacagatcctatttgacagcttattgtttcgtttagcatcatccatttccaatcttgctaccctgttaccacaattctttttctcagctgtaaaatatgccattcaaaaaaatatatcaccttacagtttttggctgaggtgaagattaatacaggttattgcttcaaaatgtaacatttgctgtattataattgccatatggggaaaacagaggagcagaaagaggagcaaatcagagaagcttactgcaaatattagtttttgtagttgtttgtttttctagatggagtctctgttgcccaggttggagtgcagtggcatgatcttggctcactgcaacctctgcctcaagcgaagcgattctcatgcctcaacctcccaagtagctggaattacaggtgtgcgccaccacacctagctactttttgtatttttagtagagatggggtttcaccatgttggccaggttggtctcaagcccctgacctcaggtgatccacccacctcggcctcccaaagtactgagattacaagcatgagccaccgcacctggccttaggttatgtttctaaagatccctttttaccaactaattttccccaatccaccctccaatctctcctctatactgccaccagaatgagtcttgcgacctgtgactaaacatactattcccatgttcaaagcacacagttgtatttgtctgggctgccctctcctccacccttgcacttgtattataattcctacccagtctttaccacccttccaccaggcacccagcagtcagagcccctcccctggacactgtgcttttagatggcccctctctggccctcctccagtgctcacccaactcctatgtcccaccttctagaacatattctgggaacctgggacccctgaatttctgttcaaatgaccatgaacccttttccagggcctggatagggctattccctaggtccatgtgggctgggagttcgcatcattttcacaaggcccttcacagaaaaagacagagctagcgggtgggaaaagaatggggacggggatggagtctccatttgtacccttatcatggcccccacaaatgtcagagccacccttgcttcaaggcctagtttaaatgccatctgtcccatgggtaacctctgatcccccagctagaatcttctacctttctgtccctaactctaatttcacactctctcgcattcaggactgtctgtcttatattagtcatgttgtcatgtcttctcccttccaatagctgttagtgccttgaaaatagatacagagctttcctcaccttcatgcctacctccccatcctaccccactcccctcctaccaccataacctagcaatttatgcaacaccttttaaatttataataaaactgtattgtttgttttggaggtgggtaaggtgggtggcggtgtgacaaacaaccccaaagtctcagtgacttacaacaataaagatttatttctactcatgttatatggttggttgtggttttgctccatggcatccaggctgcacgagcaaccccaaacataactttctcatggctgagcccatccagcaatcccaactggagtcttgctctatccccaggctggagtgcagtgttgcaatctcggctcactgcaacccctgcttcccaagttcaagcgattctcctgcttcagcctcctgagtagctgggattacagtcgtgtgccaccatgcccggcaaatttttaatttttttttagtagagatggggttttactatgttggccaggctggtctcgaactcctgaactcaagtgatctgcccgccttggcgtcccaaagtgttgggattacaggcatgagccactgcagccggtccagcaatcccttgtaaagcttctgctccatcatgatcaatgttagggctgctcgcattctattggctgatgcaagttgtatggtcaagcctggcaatggggcagggaagtatagttcctccacttacagggaggcactgccaatcacacggcagtgagtggggctatataatcctctccaagggaagggagccaatagttattaacaataatacaatggaccacaataaaatttacaatataccgactatgtgctaggcatactgctaaatgctttacctacttttttctcatttagtcctgacaattctgtcattgtccccattttacagatagggactaaggcaagcataaattctataatttgcctaggatcacataagtgaatagacaaggaatttccacctgggtaatgtaactccagagccctttgctcttatccactaagctgcaatttgtttgtgaatttattgtgccaggtcctataccagatctttcagagagagtggtacctgggaattcattacttattcattcattaatcaacatctgatgaacacctgttcactgggagtagatggggtagggaagaggcagagaagataaataagtaaataatactcaagtggggatgagtgttaagaagaataaagcaaacagaaggatgaagactctgtgtgtgtgtgtgtgtgtgtgtgtgtgtgtgtgtgtgtgtgagcaattttagtttttttttttttaagagacaaggtttcactatgttgaccaggctggagtgttgtggctattcacaggtgcgatcatagtgcactgcagcctcagactcctggcctcaagctatcctcttgcctcagcctctggagtaggtgagattacaggctcactaccacgccagacagatggtgcaattttagatattgtggtcacagacttcactgagaaggtgccatttgagtaaagacctaaagaatgtcagctccttgagggcaaggacttgtatctgttttgtttgaagttgtgtccccagcaactagaacagggcctggctcattgtaagctctcagtaataatgtgttgaacgaatgaaaggaggttagggagggaatcgtggataacttgggggaagagtgtttaaggcccaggaaacagtcagtgaaaaggctctgaggaaggagagtatctggtgagttcctgaaacaacaaagagaccagagtggctagagctgagtgagccccaggaagagaagagacagacagctcagggggatagaaggtatctctgggcccattttaaaggcttcagcttaactcagtgaaatggagagccactgaggggttttgagcagagaagtgaccagaatctgacttgtgttttcatagcatcattctggatgatgttggagaacagacagaaggaggcaagtccagaagcaggaagaccaattaggagtcccttccctcactgaaataaccaatattagtgctgggcattgtggaaactgaaatggataaattcgggaacctgcccagtacagtgaatgttaaattctgctgtgcatcttaatctcctgaaatacttaggttttaaaaatgcagatttcagaccacaccccccatcctgaaaaatcctagtttcctgggtctgggttgtgggtgttgggatc